European Patent Application EP 4 279 597 A2, published November 22, 2023. Title: NOVEL, NON-NATURALLY OCCURRING CRISPR-CAS NUCLEASES FOR GENOME EDITING. Applicant: BRAIN Biotech AG. The sequence listing filed with the application follows.

SEQUENCE LISTING (42 sequences)

SEQ ID NO: 1 - protein, 1231 aa, synthetic construct
  REGION 1..1231: note = AA Sequence of BEC85
MKSFENSCQISKTLRFGATLKEDKKKCKSHLELQEFVDISYKTLKSSATIAESLNEIELVKKCERCYSEIIKFHEAWGQIYCRTNQIAVYKDWYRQLARKARFDVGDQNSQLITLSSLSSKHNVYQGLKRSQHITNYWKDNIARQKSFLKDFSQQLKQYKRALENSDKAHTKPNLINFNKTFSILANLVNEIVIPLSNGAISFPNISKLEDGEESRHLIEFALNDYSDLVGSIGELKDAIATNGGYTPFAKVTLNHYTAEQKPHVFKNDIDAKIRELKLIELVEKLKNKTSKQIEEYFSKFDKFKIYDDRNISVIIRTQCFKYKPIPFLVKHELAKYIAEDEDAVLKVLDAIGATRSPAHDYAHNEDVFDLNHYPIKVAFDYAWEQLANSLYTTVTFPKEQCEKYLKDVFDCEVSKEPVFKFYADLLYIRKNLAVLEHKNNLPSNQEEFICKINNTFENIVLPYKISQFETYKKDILAWINDGRGHEKYTDAKQQLGFIRGGLKGRIKAQKMFRKDKYGKIKSYYENPYTKLTNEFKQISSTYGKTFAELRDKFKEKNNITKITHFGIIIEDKNRDRYLLANGLQHEQINHVSTILNKLDKSSEFITYQVKSLTSKTLIKLIKNHTTKKGAISPYADFHTSKTGFNKNEIEKNWDNYKREQVLVEYVKDCLTDSTMAKNQNWAEFGWNFEKCNSYEDIEHEIDQKSYILQKHTISKQSIASLVEGGCLLLPIINQDITSKERKDKNQFSKDWKQIFEGSKEFRLHPEFAVSYRTPIEGYPVQKRYGRLQFVCAFNCEIIPQNGEFINLKKQIENFNDEDAQKEAVEEFNKKVNHALSDKEYVVIGIDRGLKQLATLCVLDKRGKILGDFEIYKKEFVRAEKRSESHWEHTQAETRHILDLSNLRVETTIEGKKVLVDQSLTLVKKNRDTPDEEATEENKQKIKLKQLSYIRKLQHKMQTNEQDVLDLINNEPSDEEFKKRIEGLISSFGEGQKYADLPINTMREMISDLQGVIARGNNQTEKNKIIELDAADNLKQGIVANMIGIVNYIFAKYSYKAYISLEDLSRAYGGAKSGYDGRYLPSTSQDEDVDFKEQQNQMLAGLGTYQFFEMQLLKKLQKIQSDNTVLRFVPAFRSADNYRNILRLEETKYKSKPFGVVHFIDPKFTSKKCPVCSKTNVYRDKDDILVCKECGFRSDSQLKERENNIHYIHNGDDNGAYHIALKSVENLIQMK

SEQ ID NO: 2 - DNA, 3696 bp, synthetic construct
  misc_feature 1..3696: note = NT Sequence of BEC85 (Codon optimized for S. Cerevisiae)
  source 1..3696: mol_type = other DNA
atgaagtccttcgaaaactcctgccaaatttctaagactttgagattcggtgccactttgaaagaggataagaaaaagtgcaagtcccacttggaattgcaagaattcgttgacatttcctacaagaccttgaagtcatctgctaccattgctgaatccttgaacgaaatcgaattggtcaaaaagtgcgaaaggtgctactccgaaattatcaagttccatgaagcttggggtcaaatctactgtagaactaaccaaattgccgtctacaaggactggtatagacaattggctagaaaggccagattcgatgttggtgatcaaaactctcaactgatcaccttgtcatccttatcttctaagcacaacgtttaccagggtttgaagagatctcaacatattaccaactactggaaggacaacattgccagacaaaagtctttcctgaaggatttctctcaacaattgaagcagtacaagagagctttggaaaattctgataaggctcataccaagccaaacctgattaacttcaacaagaccttctccattttggccaacttggttaacgaaattgtcatcccattgtccaacggtgctatttcttttccaaacatctccaagttggaagatggtgaagaatccagacatttgattgaattcgctctgaacgattactccgatttggttggttctattggtgaattgaaggatgctattgctaccaatggtggttatactccatttgctaaggttaccttgaaccattacactgctgaacaaaagccacacgttttcaagaacgatattgatgccaagatccgtgagttgaagttgattgagttggtcgaaaagttgaagaacaagacgtccaagcaaatcgaagagtacttttccaagttcgacaagttcaagatctacgatgatagaaacatctccgttatcattagaacccaatgctttaagtacaagcccattccatttttggtcaagcacgaattggctaagtatatcgctgaagatgaagatgccgttttgaaggttttggatgcaattggtgctactagatctccagctcatgattacgctcataatgaagatgtttttgacttgaatcactacccaatcaaggttgcttttgattacgcatgggaacaattggctaactccttgtacactactgttactttcccaaaagaacagtgcgagaagtacttgaaggatgtttttgattgcgaagtctccaaagaaccagtttttaagttctacgccgacctgttgtacatcagaaagaatttggctgttttggagcacaagaacaacctgccatctaatcaagaggaattcatctgcaagattaacaacaccttcgagaacatcgttctgccatacaagatttctcaattcgaaacctacaagaaggatatcttggcctggattaacgatggtagaggtcacgaaaagtacaccgatgctaaacaacagttgggttttattagaggtggtctgaaaggtagaatcaaggctcaaaagatgttcagaaaagacaagtacggtaagatcaagtcctactacgaaaacccatacactaagttgaccaacgaattcaagcaaatctcttctacctacggtaaaaccttcgctgaattgagagacaagttcaaagaaaagaacaacatcaccaagatcacccatttcggtattatcatcgaagataagaacagggacagatacttgttggccaacggtttgcaacacgaacaaatcaaccatgtctccaccatcttgaacaagttggataagtcatccgaattcatcacctaccaagttaagtctttgacctctaagaccctgatcaagctgattaagaatcataccaccaagaagggtgcaatttctccatatgctgatttccatacttctaagaccggctttaacaaaaacgagatcgaaaagaactgggacaactacaagagagaacaagtcttggttgaatacgttaaggattgcttgaccgattctaccatggctaagaatcaaaattgggctgaatttggttggaacttcgagaagtgtaactcctacgaagatatcgaacacgaaatcgatcagaagtcttacatcttgcaaaagcataccatttccaagcaatctattgcttctttggttgaaggtggttgtttgttgttgccaattatcaaccaggacatcacctctaaagaacgtaaggacaagaatcagttctccaaggattggaagcaaatcttcgaaggttccaaagaattcagattgcatccagaattcgccgtttcttacagaactccaattgaaggttacccagtccaaaaaagatacggtagattgcaattcgtttgcgcttttaactgcgaaatcatcccacaaaatggtgagttcatcaacttgaagaagcagatcgagaacttcaacgacgaagatgctcaaaaagaagccgtcgaagagttcaacaaaaaggttaaccatgccttgtccgacaaagaatacgttgttattggtatcgacagaggcttgaagcaattagctactttgtgtgttttggacaagaggggtaagattttgggtgactttgaaatctacaaaaaagagttcgtcagagccgaaaagagatctgaatctcattgggaacatactcaagctgaaaccagacatatcttggacttgtctaacttgagagttgaaactaccattgagggcaaaaaggtgttggttgatcaatctttgacactggtcaagaagaacagagatactccagatgaagaagctaccgaagaaaacaagcagaagattaagttgaagcagctgtcctacattagaaagttgcaacacaagatgcagaccaatgaacaagatgtcttggacctgatcaacaacgaaccatctgatgaagaattcaaaaagaggatcgagggcttgatttcttcattcggtgaaggtcaaaagtacgctgatttgcctattaacaccatgagggaaatgatctctgacttgcaaggtgttattgccagaggaaacaatcagactgagaaaaacaagatcatcgaattggatgctgccgacaatttgaaacaaggtatcgttgctaacatgatcggtatcgttaactacattttcgccaagtactcctacaaggcctacatttctttagaagatttgtccagagcttacggtggtgcaaaatctggttatgatggtagatatttgccatccacctctcaagatgaggatgttgactttaaagaacagcagaatcaaatgttggctggcttgggtacttaccaattttttgaaatgcagctgctgaaaaagctgcagaagatccaatctgataacaccgttttgagatttgttccagcttttagatccgccgataactacagaaatatcttgagattggaagagactaagtacaagtctaagccattcggtgttgttcatttcatcgatccaaagttcacatctaagaagtgtccagtttgctctaagactaacgtttacagagataaggatgacatcctggtctgtaaagaatgtggttttaggtccgactcacagttgaaagaaagggaaaacaacatccactacatccacaatggtgatgataatggtgcttaccatattgccttgaagtccgtcgaaaacttgattcagatgaagtaa

SEQ ID NO: 3 - protein, 1231 aa, synthetic construct
  REGION 1..1231: note = AA Sequence of BEC67
MKSFENSCQISKTLRFGATLKEDKKKCKSHLELQEFVDISYKTLKSSATIAESLNEIELVKKCERCYSEIIKFHEAWGQIYCRTNQIAVYKDWYRQLARKARFDVGDQNSQLITLSSLSSKHNVYQGLKRSQHITNYWKDNIARQKSFLKDFSQQLKQYKRALENSDKAHTKPNLINFNKTFSILANLVNEIVIPLSNGAISFPNISKLEDGEESRHLIEFALNDYSDLVGSIGELKDAIATNGGYTPFAKVTLNHYTAEQKPHVFKNDIDAKIRELKLIELVEKLKNKTSKQIEEYFSKFDKFKIYDDRNISVIIRTQCFKYKPIPFLVKHELAKYIAEDEDAVLKVLDAIGATRSPAHDYAHNEDVFDLNHYPIKVAFDYAWEQLANSLYTTVTFPKEQCEKYLKDVFDCEVSKEPVFKFYADLLYIRKNLAVLEHKNNLPSNQEEFICKINNTFENIVLPYKISQFETYKKDILAWINDGRGHEKYTDSKRELGFIRGGLKGRIKAQKMFRKDKYGKIKSYYENPYTKLTEEFKNLAITYGKTFAELRDKFKEKNNITKITHFGIIIEDKNRDRYLLANGLQHEQINHVSTILNKLDKSSEFITYQVKSLTSKTLIKLIKNHTTKKGAISPYADFHTSKTGFNKNEIEKNWDNYKREQVLVEYVKDCLTDSTMAKNQNWAEFGWDLESCNSYEDIEHEIDQKSYILQKHTISKQSIASLVEGGCLLLPIINQDITSKERKDKNQFSKDWKQIFEGSKEFRLHPEFAVSYRTPIEGYPVQKRYGRLQFVCAFNCEIIPQNGEFINLKKQIENFNDEDAQKEAVEEFNKKVNHALSDKEYVVIGIDRGLKQLATLCVLDKRGKILGDFEIYKKEFVRAEKRSESHWEHTQAETRHILDLSNLRVETTIEGKKVLVDQSLTLVKKNRDTPDEEATEENKQKIKLKQLSYIRKLQHKMQTNEQDVLDLINNEPSDEEFKKRIEGLISSFGEGQKYADLPINTMREMISDLQGVIARGNNQTEKNKIIELDAADNLKQGIVANMIGIVNYIFAKYSYKAYISLEDLSRAYGGAKSGYDGRYLPSTSQDEDVDFKEQQNQMLAGLGTYQFFEMQLLKKLQKIQSDNTVLRFVPAFRSADNYRNILRLEETKYKSKPFGVVHFIDPKFTSKKCPVCSKTNVYRDKDDILVCKECGFRSDSQLKERENNIHYIHNGDDNGAYHIALKSVENLIQMK

SEQ ID NO: 4 - DNA, 3696 bp, synthetic construct
  misc_feature 1..3696: note = NT Sequence of BEC67 (Codon optimized for S. Cerevisiae)
  source 1..3696: mol_type = other DNA
atgaagtccttcgaaaactcctgccaaatttctaagactttgagattcggtgccactttgaaagaggataagaaaaagtgcaagtcccacttggaattgcaagaattcgttgacatttcctacaagaccttgaagtcatctgctaccattgctgaatccttgaacgaaatcgaattggtcaaaaagtgcgaaaggtgctactccgaaattatcaagttccatgaagcttggggtcaaatctactgtagaactaaccaaattgccgtctacaaggactggtatagacaattggctagaaaggccagattcgatgttggtgatcaaaactctcaactgatcaccttgtcatccttatcttctaagcacaacgtttaccagggtttgaagagatctcaacatattaccaactactggaaggacaacattgccagacaaaagtctttcctgaaggatttctctcaacaattgaagcagtacaagagagctttggaaaattctgataaggctcataccaagccaaacctgattaacttcaacaagaccttctccattttggccaacttggttaacgaaattgtcatcccattgtccaacggtgctatttcttttccaaacatctccaagttggaagatggtgaagaatccagacatttgattgaattcgctctgaacgattactccgatttggttggttctattggtgaattgaaggatgctattgctaccaatggtggttatactccatttgctaaggttaccttgaaccattacactgctgaacaaaagccacacgttttcaagaacgatattgatgccaagatccgtgagttgaagttgattgagttggtcgaaaagttgaagaacaagacgtccaagcaaatcgaagagtacttttccaagttcgacaagttcaagatctacgatgatagaaacatctccgttatcattagaacccaatgctttaagtacaagcccattccatttttggtcaagcacgaattggctaagtatatcgctgaagatgaagatgccgttttgaaggttttggatgcaattggtgctactagatctccagctcatgattacgctcataatgaagatgtttttgacttgaatcactacccaatcaaggttgcttttgattacgcatgggaacaattggctaactccttgtacactactgttactttcccaaaagaacagtgcgagaagtacttgaaggatgtttttgattgcgaagtctccaaagaaccagtttttaagttctacgccgacctgttgtacatcagaaagaatttggctgttttggagcacaagaacaacctgccatctaatcaagaggaattcatctgcaagattaacaacaccttcgagaacatcgttctgccatacaagatttctcaattcgaaacctacaagaaggatatcttggcctggattaacgatggtagaggtcacgaaaagtacaccgattctaaaagagaattgggttttattagaggtggtctgaaaggtagaatcaaggctcaaaagatgttcagaaaagacaagtacggtaagatcaagtcctactacgaaaacccatacactaagttgaccgaagagttcaagaacttggccatcacctacggtaaaaccttcgctgaattgagagacaagttcaaagaaaagaacaacatcaccaagatcacccatttcggtattatcatcgaagataagaacagggacagatacttgttggccaacggtttgcaacacgaacaaatcaaccatgtctccaccatcttgaacaagttggataagtcatccgaattcatcacctaccaagttaagtctttgacctctaagaccctgatcaagctgattaagaatcataccaccaagaagggtgcaatttctccatatgctgatttccatacttctaagaccggctttaacaaaaacgagatcgaaaagaactgggacaactacaagagagaacaagtcttggttgaatacgttaaggattgcttgaccgattctaccatggctaagaatcaaaattgggctgaatttggttgggatttggagtcttgtaactcctacgaagatatcgaacacgaaatcgatcagaagtcttacatcttgcaaaagcataccatttccaagcaatctattgcttctttggttgaaggtggttgtttgttgttgccaattatcaaccaggacatcacctctaaagaacgtaaggacaagaatcagttctccaaggattggaagcaaatcttcgaaggttccaaagaattcagattgcatccagaattcgccgtttcttacagaactccaattgaaggttacccagtccaaaaaagatacggtagattgcaattcgtttgcgcttttaactgcgaaatcatcccacaaaatggtgagttcatcaacttgaagaagcagatcgagaacttcaacgacgaagatgctcaaaaagaagccgtcgaagagttcaacaaaaaggttaaccatgccttgtccgacaaagaatacgttgttattggtatcgacagaggcttgaagcaattagctactttgtgtgttttggacaagaggggtaagattttgggtgactttgaaatctacaaaaaagagttcgtcagagccgaaaagagatctgaatctcattgggaacatactcaagctgaaaccagacatatcttggacttgtctaacttgagagttgaaactaccattgagggcaaaaaggtgttggttgatcaatctttgacactggtcaagaagaacagagatactccagatgaagaagctaccgaagaaaacaagcagaagattaagttgaagcagctgtcctacattagaaagttgcaacacaagatgcagaccaatgaacaagatgtcttggacctgatcaacaacgaaccatctgatgaagaattcaaaaagaggatcgagggcttgatttcttcattcggtgaaggtcaaaagtacgctgatttgcctattaacaccatgagggaaatgatctctgacttgcaaggtgttattgccagaggaaacaatcagactgagaaaaacaagatcatcgaattggatgctgccgacaatttgaaacaaggtatcgttgctaacatgatcggtatcgttaactacattttcgccaagtactcctacaaggcctacatttctttagaagatttgtccagagcttacggtggtgcaaaatctggttatgatggtagatatttgccatccacctctcaagatgaggatgttgactttaaagaacagcagaatcaaatgttggctggcttgggtacttaccaattttttgaaatgcagctgctgaaaaagctgcagaagatccaatctgataacaccgttttgagatttgttccagcttttagatccgccgataactacagaaatatcttgagattggaagagactaagtacaagtctaagccattcggtgttgttcatttcatcgatccaaagttcacatctaagaagtgtccagtttgctctaagactaacgtttacagagataaggatgacatcctggtctgtaaagaatgtggttttaggtccgactcacagttgaaagaaagggaaaacaacatccactacatccacaatggtgatgataatggtgcttaccatattgccttgaagtccgtcgaaaacttgattcagatgaagtaa

SEQ ID NO: 5 - protein, 7 aa, synthetic construct
  REGION 1..7: note = RuvC I AA Sequence of BEC85, BEC67 and BEC10
IGIDRGL

SEQ ID NO: 6 - protein, 7 aa, synthetic construct
  REGION 1..7: note = RuvC II AA Sequence of BEC85, BEC67 and BEC10
ISLEDLS

SEQ ID NO: 7 - protein, 7 aa, synthetic construct
  REGION 1..7: note = RuvC II AA Sequence of BEC85, BEC67 and BEC10
HNGDDNG

SEQ ID NO: 8 - DNA, 19 bp, synthetic construct
  misc_feature 1..19: note = Stem-Loop Consensus Sequence
  variation 1: note = /replace="a,c,g,t"
  variation 11: note = /replace="a,c,g,t"
  source 1..19: mol_type = other DNA
natttctactnttgtagat

SEQ ID NO: 9 - DNA, 19 bp, synthetic construct
  misc_feature 1..19: note = BEC85 Stem-Loop Sequence
  source 1..19: mol_type = other DNA
aatttctactgttgtagat

SEQ ID NO: 10 - DNA, 19 bp, synthetic construct
  misc_feature 1..19: note = BEC67 and BEC10 Stem-Loop Sequence
  source 1..19: mol_type = other DNA
gatttctactattgtagat

SEQ ID NO: 11 - DNA, 27 bp, synthetic construct
  misc_feature 1..27: note = Nuclear Localization Tag
  source 1..27: mol_type = other DNA
atggctcccaaaaagaaaaggaaggtg

SEQ ID NO: 12 - DNA, 582 bp, synthetic construct
  misc_feature 1..582: note = Tpi1 Promotor Sequence
  source 1..582: mol_type = other DNA
gtttaaagattacggatatttaacttacttagaataatgccatttttttgagttataataatcctacgttagtgtgagcgggatttaaactgtgaggaccttaatacattcagacacttctgcggtatcaccctacttattcccttcgagattatatctaggaacccatcaggttggtggaagattacccgttctaagacttttcagcttcctctattgatgttacacctggacaccccttttctggcatccagtttttaatcttcagtggcatgtgagattctccgaaattaattaaagcaatcacacaatgctctcggataccacctcggttgaaactgacaggtggtttgttacgcatgctaatgcaaaggagcctatatacctttggctcggctgctgtaacagggaatataaagggcagcataatttaggagtttagtgaacttgcaacatttactattttcccttcttacgtaaatatttttctttttaattctaaatcaatctttttcaattttttgtttgtattcttttcttgcttaaatctataactacaaaaaacacatacataaactaaaa

SEQ ID NO: 13 - DNA, 191 bp, synthetic construct
  misc_feature 1..191: note = Cps1 Terminator
  source 1..191: mol_type = other DNA
gcgcaatgattgaatagtcaaagattttttttttttaattttttttttttaattttttttttttttcatagaactttttatttaaataaatcacgtctatatatgtatcagtataacgtaaaaaaaaaaacaccgtcagttaaacaaaacataaataaaaaaaaaaagaagtgtcaaatcaagtgtcaaat

SEQ ID NO: 14 - DNA, 67 bp, synthetic construct
  misc_feature 1..67: note = Em7 Promotor
  source 1..67: mol_type = other DNA
gtgttgacaattaatcatcggcatagtatatcggcatagtataatacgacaaggtgaggaactaaac

SEQ ID NO: 15 - DNA, 514 bp, synthetic construct
  misc_feature 1..514: note = CEN6 Centromere
  source 1..514: mol_type = other DNA
ggtccttttcatcacgtgctataaaaataattataatttaaattttttaatataaatatataaattaaaaatagaaagtaaaaaaagaaattaaagaaaaaatagtttttgttttccgaagatgtaaaagactctagggggatcgccaacaaatactaccttttatcttgctcttcctgctctcaggtattaatgccgaattgtttcatcttgtctgtgtagaagaccacacacgaaaatcctgtgattttacattttacttatcgttaatcgaatgtatatctatttaatctgcttttcttgtctaataaatatatatgtaaagtacgctttttgttgaaattttttaaacctttgtttatttttttttcttcattccgtaactcttctaccttctttatttactttctaaaatccaaatacaaaacataaaaataaataaacacagagtaaattcccaaattattccatcattaaaagatacgaggcgcgtgtaagttacaggcaagcgatc

SEQ ID NO: 16 - DNA, 810 bp, synthetic construct
  misc_feature 1..810: note = kanMX Marker Gene
  source 1..810: mol_type = other DNA
atgggtaaggaaaagactcacgtttcgaggccgcgattaaattccaacatggatgctgatttatatgggtataaatgggctcgcgataatgtcgggcaatcaggtgcgacaatctatcgattgtatgggaagcccgatgcgccagagttgtttctgaaacatggcaaaggtagcgttgccaatgatgttacagatgagatggtcagactaaactggctgacggaatttatgcctcttccgaccatcaagcattttatccgtactcctgatgatgcatggttactcaccactgcgatccccggcaaaacagcattccaggtattagaagaatatcctgattcaggtgaaaatattgttgatgcgctggcagtgttcctgcgccggttgcattcgattcctgtttgtaattgtccttttaacagcgatcgcgtatttcgcctcgctcaggcgcaatcacgaatgaataacggtttggttgatgcgagtgattttgatgacgagcgtaatggctggcctgttgaacaagtctggaaagaaatgcataagcttttgccattctcaccggattcagtcgtcactcatggtgatttctcacttgataaccttatttttgacgaggggaaattaataggttgtattgatgttggacgagtcggaatcgcagaccgataccaggatcttgccatcctatggaactgcctcggtgagttttctccttcattacagaaacggctttttcaaaaatatggtattgataatcctgatatgaataaattgcagtttcatttgatgctcgatgagtttttctaa

SEQ ID NO: 17 - DNA, 412 bp, synthetic construct
  misc_feature 1..412: note = Tef1 Promotor Sequence
  source 1..412: mol_type = other DNA
gcccttagattagattgctatgctttctttctaatgagcaagaagtaaaaaaagttgtaatagaacaagaaaaatgaaactgaaacttgagaaattgaagaccgtttattaacttaaatatcaatgggaggtcatcgaaagagaaaaaaatcaaaaaaaaaaattttcaagaaaaagaaacgtgataaaaatttttattgcctttttcgacgaagaaaaagaaacgaggcggtctcttttttcttttccaaacctttagtacgggtaattaacgacaccctagaggaagaaagaggggaaatttagtatgctgtgcttgggtgttttgaagtggtacggcgatgcgcggagtccgagaaaatctggaagagtaaaaaaggagtagaaacattttgaagctatggtgtgtggg

SEQ ID NO: 18 - DNA, 281 bp, synthetic construct
  misc_feature 1..281: note = SNR52 RNA Polymerase III Promotor
  source 1..281: mol_type = other DNA
ctgcatctgcggatcctctttgaaaagataatgtatgattatgctttcactcatatttatacagaaacttgatgttttctttcgagtatatacaaggtgattacatgtacgtttgaagtacaactctagattttgtagtgccctcttgggctagcggtaaaggtgcgcattttttcacaccctacaatgttctgttcaaaagattttggtcaaacgctgtagaagtgaaagttggtgcgcatgtttcggcgttcgaaacttctccgcagtgaaagataaat

SEQ ID NO: 19 - DNA, 20 bp, synthetic construct
  misc_feature 1..20: note = SUP4 Terminator Sequence
  source 1..20: mol_type = other DNA
tttttttgttttttatgtct

SEQ ID NO: 20 - DNA, 24 bp, synthetic construct
  misc_feature 1..24: note = BEC85, BEC67, BEC10, SuCms1 and SeqID63 Ade2 Spacer Sequence
  source 1..24: mol_type = other DNA
gtgtaggaacatcaacatgctcaa

SEQ ID NO: 21 - DNA, 8269 bp, synthetic construct
  misc_feature 1..8269: note = CRISPR/BEC85 vector system
  source 1..8269: mol_type = other DNA
agcttgcaaattaaagccttcgagcgtcccaaaaccttctcaagcaaggttttcagtataatgttacatgcgtacacgcgtctgtacagaaaaaaaagaaaaatttgaaatataaataacgttcttaatactaacataactataaaaaaataaatagggacctagacttcaggttgtctaactccttccttttcggttagagcggatgtggggggagggcgtgaatgtaagcgtgacataactaattacatgatatcgacaaaggaaaagggggacggatctccgaggcctcggacccgtcgggccgcgtcggacgtgtcagtcctgctcctcgcaattgttagaaaaactcatcgagcatcaaatgaaactgcaatttattcatatcaggattatcaataccatatttttgaaaaagccgtttctgtaatgaaggagaaaactcaccgaggcagttccataggatggcaagatcctggtatcggtctgcgattccgactcgtccaacatcaatacaacctattaatttcccctcgtcaaaaataaggttatcaagtgagaaatcaccatgagtgacgactgaatccggtgagaatggcaaaagcttatgcatttctttccagacttgttcaacaggccagccattacgctcgtcatcaaaatcactcgcatcaaccaaaccgttattcattcgtgattgcgcctgagcgaggcgaaatacgcgatcgctgttaaaaggacaattacaaacaggaatcgaatgcaaccggcgcaggaacactgccagcgcatcaacaatattttcacctgaatcaggatattcttctaatacctggaatgctgttttgccggggatcgcagtggtgagtaaccatgcatcatcaggagtacggataaaatgcttgatggtcggaagaggcataaattccgtcagccagtttagtctgaccatctcatctgtaacatcattggcaacgctacctttgccatgtttcagaaacaactctggcgcatcgggcttcccatacaatcgatagattgtcgcacctgattgcccgacattatcgcgagcccatttatacccatataaatcagcatccatgttggaatttaatcgcggcctcgaaacgtgagtcttttccttacccatggtttagttcctcaccttgtcgtattatactatgccgatatactatgccgatgattaattgtcaacaccgcccttagattagattgctatgctttctttctaatgagcaagaagtaaaaaaagttgtaatagaacaagaaaaatgaaactgaaacttgagaaattgaagaccgtttattaacttaaatatcaatgggaggtcatcgaaagagaaaaaaatcaaaaaaaaaaattttcaagaaaaagaaacgtgataaaaatttttattgcctttttcgacgaagaaaaagaaacgaggcggtctcttttttcttttccaaacctttagtacgggtaattaacgacaccctagaggaagaaagaggggaaatttagtatgctgtgcttgggtgttttgaagtggtacggcgatgcgcggagtccgagaaaatctggaagagtaaaaaaggagtagaaacattttgaagctatggtgtgtgggggatccgcacaaacgaaggtctcactgatcgcttgcctgtaacttacacgcgcctcgtatcttttaatgatggaataatttgggaatttactctgtgtttatttatttttatgttttgtatttggattttagaaagtaaataaagaaggtagaagagttacggaatgaagaaaaaaaaataaacaaaggtttaaaaaatttcaacaaaaagcgtactttacatatatatttattagacaagaaaagcagattaaatagatatacattcgattaacgataagtaaaatgtaaaatcacaggattttcgtgtgtggtcttctacacagacaagatgaaacaattcggcattaatacctgagagcaggaagagcaagataaaaggtagtatttgttggcgatccccctagagtcttttacatcttcggaaaacaaaaactattttttctttaatttctttttttactttctatttttaatttatatatttatattaaaaaatttaaattataattatttttatagcacgtgatgaaaaggacccatcgataagctggtaccgagctcggatcccggtctgcatctgcggatcctctttgaaaagataatgtatgattatgctttcactcatatttatacagaaacttgatgttttctttcgagtatatacaaggtgattacatgtacgtttgaagtacaactctagattttgtagtgccctcttgggctagcggtaaaggtgcgcattttttcacaccctacaatgttctgttcaaaagattttggtcaaacgctgtagaagtgaaagttggtgcgcatgtttcggcgttcgaaacttctccgcagtgaaagataaatgatcgaatttctactgttgtagatgtgtaggaacatcaacatgctcaatttttttgttttttatgtctcctgcaggtttaaagattacggatatttaacttacttagaataatgccatttttttgagttataataatcctacgttagtgtgagcgggatttaaactgtgaggaccttaatacattcagacacttctgcggtatcaccctacttattcccttcgagattatatctaggaacccatcaggttggtggaagattacccgttctaagacttttcagcttcctctattgatgttacacctggacaccccttttctggcatccagtttttaatcttcagtggcatgtgagattctccgaaattaattaaagcaatcacacaatgctctcggataccacctcggttgaaactgacaggtggtttgttacgcatgctaatgcaaaggagcctatatacctttggctcggctgctgtaacagggaatataaagggcagcataatttaggagtttagtgaacttgcaacatttactattttcccttcttacgtaaatatttttctttttaattctaaatcaatctttttcaattttttgtttgtattcttttcttgcttaaatctataactacaaaaaacacatacataaactaaaaatggctcccaaaaagaaaaggaaggtgatgaagtccttcgaaaactcctgccaaatttctaagactttgagattcggtgccactttgaaagaggataagaaaaagtgcaagtcccacttggaattgcaagaattcgttgacatttcctacaagaccttgaagtcatctgctaccattgctgaatccttgaacgaaatcgaattggtcaaaaagtgcgaaaggtgctactccgaaattatcaagttccatgaagcttggggtcaaatctactgtagaactaaccaaattgccgtctacaaggactggtatagacaattggctagaaaggccagattcgatgttggtgatcaaaactctcaactgatcaccttgtcatccttatcttctaagcacaacgtttaccagggtttgaagagatctcaacatattaccaactactggaaggacaacattgccagacaaaagtctttcctgaaggatttctctcaacaattgaagcagtacaagagagctttggaaaattctgataaggctcataccaagccaaacctgattaacttcaacaagaccttctccattttggccaacttggttaacgaaattgtcatcccattgtccaacggtgctatttcttttccaaacatctccaagttggaagatggtgaagaatccagacatttgattgaattcgctctgaacgattactccgatttggttggttctattggtgaattgaaggatgctattgctaccaatggtggttatactccatttgctaaggttaccttgaaccattacactgctgaacaaaagccacacgttttcaagaacgatattgatgccaagatccgtgagttgaagttgattgagttggtcgaaaagttgaagaacaagacgtccaagcaaatcgaagagtacttttccaagttcgacaagttcaagatctacgatgatagaaacatctccgttatcattagaacccaatgctttaagtacaagcccattccatttttggtcaagcacgaattggctaagtatatcgctgaagatgaagatgccgttttgaaggttttggatgcaattggtgctactagatctccagctcatgattacgctcataatgaagatgtttttgacttgaatcactacccaatcaaggttgcttttgattacgcatgggaacaattggctaactccttgtacactactgttactttcccaaaagaacagtgcgagaagtacttgaaggatgtttttgattgcgaagtctccaaagaaccagtttttaagttctacgccgacctgttgtacatcagaaagaatttggctgttttggagcacaagaacaacctgccatctaatcaagaggaattcatctgcaagattaacaacaccttcgagaacatcgttctgccatacaagatttctcaattcgaaacctacaagaaggatatcttggcctggattaacgatggtagaggtcacgaaaagtacaccgatgctaaacaacagttgggttttattagaggtggtctgaaaggtagaatcaaggctcaaaagatgttcagaaaagacaagtacggtaagatcaagtcctactacgaaaacccatacactaagttgaccaacgaattcaagcaaatctcttctacctacggtaaaaccttcgctgaattgagagacaagttcaaagaaaagaacaacatcaccaagatcacccatttcggtattatcatcgaagataagaacagggacagatacttgttggccaacggtttgcaacacgaacaaatcaaccatgtctccaccatcttgaacaagttggataagtcatccgaattcatcacctaccaagttaagtctttgacctctaagaccctgatcaagctgattaagaatcataccaccaagaagggtgcaatttctccatatgctgatttccatacttctaagaccggctttaacaaaaacgagatcgaaaagaactgggacaactacaagagagaacaagtcttggttgaatacgttaaggattgcttgaccgattctaccatggctaagaatcaaaattgggctgaatttggttggaacttcgagaagtgtaactcctacgaagatatcgaacacgaaatcgatcagaagtcttacatcttgcaaaagcataccatttccaagcaatctattgcttctttggttgaaggtggttgtttgttgttgccaattatcaaccaggacatcacctctaaagaacgtaaggacaagaatcagttctccaaggattggaagcaaatcttcgaaggttccaaagaattcagattgcatccagaattcgccgtttcttacagaactccaattgaaggttacccagtccaaaaaagatacggtagattgcaattcgtttgcgcttttaactgcgaaatcatcccacaaaatggtgagttcatcaacttgaagaagcagatcgagaacttcaacgacgaagatgctcaaaaagaagccgtcgaagagttcaacaaaaaggttaaccatgccttgtccgacaaagaatacgttgttattggtatcgacagaggcttgaagcaattagctactttgtgtgttttggacaagaggggtaagattttgggtgactttgaaatctacaaaaaagagttcgtcagagccgaaaagagatctgaatctcattgggaacatactcaagctgaaaccagacatatcttggacttgtctaacttgagagttgaaactaccattgagggcaaaaaggtgttggttgatcaatctttgacactggtcaagaagaacagagatactccagatgaagaagctaccgaagaaaacaagcagaagattaagttgaagcagctgtcctacattagaaagttgcaacacaagatgcagaccaatgaacaagatgtcttggacctgatcaacaacgaaccatctgatgaagaattcaaaaagaggatcgagggcttgatttcttcattcggtgaaggtcaaaagtacgctgatttgcctattaacaccatgagggaaatgatctctgacttgcaaggtgttattgccagaggaaacaatcagactgagaaaaacaagatcatcgaattggatgctgccgacaatttgaaacaaggtatcgttgctaacatgatcggtatcgttaactacattttcgccaagtactcctacaaggcctacatttctttagaagatttgtccagagcttacggtggtgcaaaatctggttatgatggtagatatttgccatccacctctcaagatgaggatgttgactttaaagaacagcagaatcaaatgttggctggcttgggtacttaccaattttttgaaatgcagctgctgaaaaagctgcagaagatccaatctgataacaccgttttgagatttgttccagcttttagatccgccgataactacagaaatatcttgagattggaagagactaagtacaagtctaagccattcggtgttgttcatttcatcgatccaaagttcacatctaagaagtgtccagtttgctctaagactaacgtttacagagataaggatgacatcctggtctgtaaagaatgtggttttaggtccgactcacagttgaaagaaagggaaaacaacatccactacatccacaatggtgatgataatggtgcttaccatattgccttgaagtccgtcgaaaacttgattcagatgaagtaagcggccgcaatgccggcgcaatgattgaatagtcaaagattttttttttttaattttttttttttaattttttttttttttcatagaactttttatttaaataaatcacgtctatatatgtatcagtataacgtaaaaaaaaaaacaccgtcagttaaacaaaacataaataaaaaaaaaaagaagtgtcaaatcaagtgtcaaatggccctgcattaatgaatcggccaacgcgcggggagaggcggtttgcgtattgggcgctcttccgcttcctcgctcactgactcgctgcgctcggtcgttcggctgcggcgagcggtatcagctcactcaaaggcggtaatacggttatccacagaatcaggggataacgcaggaaagaacatgtgagcaaaaggccagcaaaaggccaggaaccgtaaaaaggccgcgttgctggcgtttttccataggctccgcccccctgacgagcatcacaaaaatcgacgctcaagtcagaggtggcgaaacccgacaggactataaagataccaggcgtttccccctggaagctccctcgtgcgctctcctgttccgaccctgccgcttaccggatacctgtccgcctttctcccttcgggaagcgtggcgctttctcatagctcacgctgtaggtatctcagttcggtgtaggtcgttcgctccaagctgggctgtgtgcacgaaccccccgttcagcccgaccgctgcgccttatccggtaactatcgtcttgagtccaacccggtaagacacgacttatcgccactggcagcagccactggtaacaggattagcagagcgaggtatgtaggcggtgctacagagttcttgaagtggtggcctaactacggctacactagaagaacagtatttggtatctgcgctctgctgaagccagttaccttcggaaaaagagttggtagctcttgatccggcaaacaaaccaccgctggtagcggtggtttttttgtttgcaagcagcagattacgcgcagaaaaaaaggatctcaagaagatcctttgatcttttctacggggtctgacgctcagtggaacgaaaactcacgttaagggattttggtcatgagattatcaaaaaggatcttcacctagatccttttaaattaaaaatgaagttttaaatcaatctaaagtatatatgagtaaacttggtctgacagttaccaatgcttaatcagtgaggcacctatctcagcgatctgtctatttcgttcatccatagttgcctgactccccgtcgtgtagataactacgatacgggagggcttaccatctggccccagtgctgcaatgataccgcgagacccacgctcaccggctccagatttatcagcaataaaccagccagccggaagggc

SEQ ID NO: 22 - DNA, 8269 bp, synthetic construct
  misc_feature 1..8269: note = CRISPR/BEC67 vector system
  source 1..8269: mol_type = other DNA
agcttgcaaattaaagccttcgagcgtcccaaaaccttctcaagcaaggttttcagtataatgttacatgcgtacacgcgtctgtacagaaaaaaaagaaaaatttgaaatataaataacgttcttaatactaacataactataaaaaaataaatagggacctagacttcaggttgtctaactccttccttttcggttagagcggatgtggggggagggcgtgaatgtaagcgtgacataactaattacatgatatcgacaaaggaaaagggggacggatctccgaggcctcggacccgtcgggccgcgtcggacgtgtcagtcctgctcctcgcaattgttagaaaaactcatcgagcatcaaatgaaactgcaatttattcatatcaggattatcaataccatatttttgaaaaagccgtttctgtaatgaaggagaaaactcaccgaggcagttccataggatggcaagatcctggtatcggtctgcgattccgactcgtccaacatcaatacaacctattaatttcccctcgtcaaaaataaggttatcaagtgagaaatcaccatgagtgacgactgaatccggtgagaatggcaaaagcttatgcatttctttccagacttgttcaacaggccagccattacgctcgtcatcaaaatcactcgcatcaaccaaaccgttattcattcgtgattgcgcctgagcgaggcgaaatacgcgatcgctgttaaaaggacaattacaaacaggaatcgaatgcaaccggcgcaggaacactgccagcgcatcaacaatattttcacctgaatcaggatattcttctaatacctggaatgctgttttgccggggatcgcagtggtgagtaaccatgcatcatcaggagtacggataaaatgcttgatggtcggaagaggcataaattccgtcagccagtttagtctgaccatctcatctgtaacatcattggcaacgctacctttgccatgtttcagaaacaactctggcgcatcgggcttcccatacaatcgatagattgtcgcacctgattgcccgacattatcgcgagcccatttatacccatataaatcagcatccatgttggaatttaatcgcggcctcgaaacgtgagtcttttccttacccatggtttagttcctcaccttgtcgtattatactatgccgatatactatgccgatgattaattgtcaacaccgcccttagattagattgctatgctttctttctaatgagcaagaagtaaaaaaagttgtaatagaacaagaaaaatgaaactgaaacttgagaaattgaagaccgtttattaacttaaatatcaatgggaggtcatcgaaagagaaaaaaatcaaaaaaaaaaattttcaagaaaaagaaacgtgataaaaatttttattgcctttttcgacgaagaaaaagaaacgaggcggtctcttttttcttttccaaacctttagtacgggtaattaacgacaccctagaggaagaaagaggggaaatttagtatgctgtgcttgggtgttttgaagtggtacggcgatgcgcggagtccgagaaaatctggaagagtaaaaaaggagtagaaacattttgaagctatggtgtgtgggggatccgcacaaacgaaggtctcactgatcgcttgcctgtaacttacacgcgcctcgtatcttttaatgatggaataatttgggaatttactctgtgtttatttatttttatgttttgtatttggattttagaaagtaaataaagaaggtagaagagttacggaatgaagaaaaaaaaataaacaaaggtttaaaaaatttcaacaaaaagcgtactttacatatatatttattagacaagaaaagcagattaaatagatatacattcgattaacgataagtaaaatgtaaaatcacaggattttcgtgtgtggtcttctacacagacaagatgaaacaattcggcattaatacctgagagcaggaagagcaagataaaaggtagtatttgttggcgatccccctagagtcttttacatcttcggaaaacaaaaactattttttctttaatttctttttttactttctatttttaatttatatatttatattaaaaaatttaaattataattatttttatagcacgtgatgaaaaggacccatcgataagctggtaccgagctcggatcccggtctgcatctgcggatcctctttgaaaagataatgtatgattatgctttcactcatatttatacagaaacttgatgttttctttcgagtatatacaaggtgattacatgtacgtttgaagtacaactctagattttgtagtgccctcttgggctagcggtaaaggtgcgcattttttcacaccctacaatgttctgttcaaaagattttggtcaaacgctgtagaagtgaaagttggtgcgcatgtttcggcgttcgaaacttctccgcagtgaaagataaatgatcgaatttctactgttgtagatgtgtaggaacatcaacatgctcaatttttttgttttttatgtctcctgcaggtttaaagattacggatatttaacttacttagaataatgccatttttttgagttataataatcctacgttagtgtgagcgggatttaaactgtgaggaccttaatacattcagacacttctgcggtatcaccctacttattcccttcgagattatatctaggaacccatcaggttggtggaagattacccgttctaagacttttcagcttcctctattgatgttacacctggacaccccttttctggcatccagtttttaatcttcagtggcatgtgagattctccgaaattaattaaagcaatcacacaatgctctcggataccacctcggttgaaactgacaggtggtttgttacgcatgctaatgcaaaggagcctatatacctttggctcggctgctgtaacagggaatataaagggcagcataatttaggagtttagtgaacttgcaacatttactattttcccttcttacgtaaatatttttctttttaattctaaatcaatctttttcaattttttgtttgtattcttttcttgcttaaatctataactacaaaaaacacatacataaactaaaaatggctcccaaaaagaaaaggaaggtgatgaagtccttcgaaaactcctgccaaatttctaagactttgagattcggtgccactttgaaagaggataagaaaaagtgcaagtcccacttggaattgcaagaattcgttgacatttcctacaagaccttgaagtcatctgctaccattgctgaatccttgaacgaaatcgaattggtcaaaaagtgcgaaaggtgctactccgaaattatcaagttccatgaagcttggggtcaaatctactgtagaactaaccaaattgccgtctacaaggactggtatagacaattggctagaaaggccagattcgatgttggtgatcaaaactctcaactgatcaccttgtcatccttatcttctaagcacaacgtttaccagggtttgaagagatctcaacatattaccaactactggaaggacaacattgccagacaaaagtctttcctgaaggatttctctcaacaattgaagcagtacaagagagctttggaaaattctgataaggctcataccaagccaaacctgattaacttcaacaagaccttctccattttggccaacttggttaacgaaattgtcatcccattgtccaacggtgctatttcttttccaaacatctccaagttggaagatggtgaagaatccagacatttgattgaattcgctctgaacgattactccgatttggttggttctattggtgaattgaaggatgctattgctaccaatggtggttatactccatttgctaaggttaccttgaaccattacactgctgaacaaaagccacacgttttcaagaacgatattgatgccaagatccgtgagttgaagttgattgagttggtcgaaaagttgaagaacaagacgtccaagcaaatcgaagagtacttttccaagttcgacaagttcaagatctacgatgatagaaacatctccgttatcattagaacccaatgctttaagtacaagcccattccatttttggtcaagcacgaattggctaagtatatcgctgaagatgaagatgccgttttgaaggttttggatgcaattggtgctactagatctccagctcatgattacgctcataatgaagatgtttttgacttgaatcactacccaatcaaggttgcttttgattacgcatgggaacaattggctaactccttgtacactactgttactttcccaaaagaacagtgcgagaagtacttgaaggatgtttttgattgcgaagtctccaaagaaccagtttttaagttctacgccgacctgttgtacatcagaaagaatttggctgttttggagcacaagaacaacctgccatctaatcaagaggaattcatctgcaagattaacaacaccttcgagaacatcgttctgccatacaagatttctcaattcgaaacctacaagaaggatatcttggcctggattaacgatggtagaggtcacgaaaagtacaccgattctaaaagagaattgggttttattagaggtggtctgaaaggtagaatcaaggctcaaaagatgttcagaaaagacaagtacggtaagatcaagtcctactacgaaaacccatacactaagttgaccgaagagttcaagaacttggccatcacctacggtaaaaccttcgctgaattgagagacaagttcaaagaaaagaacaacatcaccaagatcacccatttcggtattatcatcgaagataagaacagggacagatacttgttggccaacggtttgcaacacgaacaaatcaaccatgtctccaccatcttgaacaagttggataagtcatccgaattcatcacctaccaagttaagtctttgacctctaagaccctgatcaagctgattaagaatcataccaccaagaagggtgcaatttctccatatgctgatttccatacttctaagaccggctttaacaaaaacgagatcgaaaagaactgggacaactacaagagagaacaagtcttggttgaatacgttaaggattgcttgaccgattctaccatggctaagaatcaaaattgggctgaatttggttgggatttggagtcttgtaactcctacgaagatatcgaacacgaaatcgatcagaagtcttacatcttgcaaaagcataccatttccaagcaatctattgcttctttggttgaaggtggttgtttgttgttgccaattatcaaccaggacatcacctctaaagaacgtaaggacaagaatcagttctccaaggattggaagcaaatcttcgaaggttccaaagaattcagattgcatccagaattcgccgtttcttacagaactccaattgaaggttacccagtccaaaaaagatacggtagattgcaattcgtttgcgcttttaactgcgaaatcatcccacaaaatggtgagttcatcaacttgaagaagcagatcgagaacttcaacgacgaagatgctcaaaaagaagccgtcgaagagttcaacaaaaaggttaaccatgccttgtccgacaaagaatacgttgttattggtatcgacagaggcttgaagcaattagctactttgtgtgttttggacaagaggggtaagattttgggtgactttgaaatctacaaaaaagagttcgtcagagccgaaaagagatctgaatctcattgggaacatactcaagctgaaaccagacatatcttggacttgtctaacttgagagttgaaactaccattgagggcaaaaaggtgttggttgatcaatctttgacactggtcaagaagaacagagatactccagatgaagaagctaccgaagaaaacaagcagaagattaagttgaagcagctgtcctacattagaaagttgcaacacaagatgcagaccaatgaacaagatgtcttggacctgatcaacaacgaaccatctgatgaagaattcaaaaagaggatcgagggcttgatttcttcattcggtgaaggtcaaaagtacgctgatttgcctattaacaccatgagggaaatgatctctgacttgcaaggtgttattgccagaggaaacaatcagactgagaaaaacaagatcatcgaattggatgctgccgacaatttgaaacaaggtatcgttgctaacatgatcggtatcgttaactacattttcgccaagtactcctacaaggcctacatttctttagaagatttgtccagagcttacggtggtgcaaaatctggttatgatggtagatatttgccatccacctctcaagatgaggatgttgactttaaagaacagcagaatcaaatgttggctggcttgggtacttaccaattttttgaaatgcagctgctgaaaaagctgcagaagatccaatctgataacaccgttttgagatttgttccagcttttagatccgccgataactacagaaatatcttgagattggaagagactaagtacaagtctaagccattcggtgttgttcatttcatcgatccaaagttcacatctaagaagtgtccagtttgctctaagactaacgtttacagagataaggatgacatcctggtctgtaaagaatgtggttttaggtccgactcacagttgaaagaaagggaaaacaacatccactacatccacaatggtgatgataatggtgcttaccatattgccttgaagtccgtcgaaaacttgattcagatgaagtaagcggccgcaatgccggcgcaatgattgaatagtcaaagattttttttttttaattttttttttttaattttttttttttttcatagaactttttatttaaataaatcacgtctatatatgtatcagtataacgtaaaaaaaaaaacaccgtcagttaaacaaaacataaataaaaaaaaaaagaagtgtcaaatcaagtgtcaaatggccctgcattaatgaatcggccaacgcgcggggagaggcggtttgcgtattgggcgctcttccgcttcctcgctcactgactcgctgcgctcggtcgttcggctgcggcgagcggtatcagctcactcaaaggcggtaatacggttatccacagaatcaggggataacgcaggaaagaacatgtgagcaaaaggccagcaaaaggccaggaaccgtaaaaaggccgcgttgctggcgtttttccataggctccgcccccctgacgagcatcacaaaaatcgacgctcaagtcagaggtggcgaaacccgacaggactataaagataccaggcgtttccccctggaagctccctcgtgcgctctcctgttccgaccctgccgcttaccggatacctgtccgcctttctcccttcgggaagcgtggcgctttctcatagctcacgctgtaggtatctcagttcggtgtaggtcgttcgctccaagctgggctgtgtgcacgaaccccccgttcagcccgaccgctgcgccttatccggtaactatcgtcttgagtccaacccggtaagacacgacttatcgccactggcagcagccactggtaacaggattagcagagcgaggtatgtaggcggtgctacagagttcttgaagtggtggcctaactacggctacactagaagaacagtatttggtatctgcgctctgctgaagccagttaccttcggaaaaagagttggtagctcttgatccggcaaacaaaccaccgctggtagcggtggtttttttgtttgcaagcagcagattacgcgcagaaaaaaaggatctcaagaagatcctttgatcttttctacggggtctgacgctcagtggaacgaaaactcacgttaagggattttggtcatgagattatcaaaaaggatcttcacctagatccttttaaattaaaaatgaagttttaaatcaatctaaagtatatatgagtaaacttggtctgacagttaccaatgcttaatcagtgaggcacctatctcagcgatctgtctatttcgttcatccatagttgcctgactccccgtcgtgtagataactacgatacgggagggcttaccatctggccccagtgctgcaatgataccgcgagacccacgctcaccggctccagatttatcagcaataaaccagccagccggaagggc

SEQ ID NO: 23 - DNA, 838 bp, synthetic construct
  misc_feature 1..838: note = Ade2 HDR-template for BEC85, BEC67, BEC10, SuCms1 and SeqID63
  source 1..838: mol_type = other DNA
ttgttgcatggctacgaaccgggtaatactaagtgattgactcttgctgaccttttattaagaactaaatggacaatattatggagcatttcatgtataaattggtgcgtaaaatcgttggatctctcttctaagtacatcctactataacaatcaagaaaaacaagaaaatcggacaaaacaatcaagtatggattctagaacagttggtatattaggagggggacaattgggacgtatgattgttgaggcagcaaacaggctcaacattaagacggtaatactagatgctgaaaattctcctgccaaacaaataagcaactccaatgaccacgttaatggctccttttccaatcctcttgatatcgaaaaactagctgaaaaatgtgatgtgctaacgattgagaattcttcaagtaaaacatcccaaattaaaaatttacccttctccagaaacaatcagattgatacaagacaaatatattcaaaaagagcatttaatcaaaaatggtatagcagttacccaaagtgttcctgtggaacaagccagtgagacgtccctattgaatgttggaagagatttgggttttccattcgtcttgaagtcgaggactttggcatacgatggaagaggtaacttcgttgtaaagaataaggaaatgattccggaagctttggaagtactgaaggatcgtcctttgtacgccgaaaaatgggcaccatttactaaagaattagcagtcatgattgtgagatctgttaacggtttagtgttttcttacccaattgtagagactatccacaaggacaatatttgtgacttatgttatgcgcctgc

SEQ ID NO: 24 - DNA, 4107 bp, synthetic construct
  misc_feature 1..4107: note = Codon Optimized SpCas9 Sequence for S.cerevisiae
  source 1..4107: mol_type = other DNA
atggacaagaagtactccatcggtttggatattggtacaaattctgttggttgggccgttattactgatgagtacaaagttccatccaagaagttcaaggttttgggtaacactgataggcactccatcaaaaagaatttgattggtgccttgttgttcgactctggtgaaactgctgaagctactagattgaaaagaaccgctagaagaagatacaccagaagaaagaacagaatctgctacttgcaagagatcttctctaacgaaatggccaaggttgatgattcattcttccacagattggaagagtccttcttggttgaagaggataagaaacacgaaagacatccaatcttcggtaacatcgttgatgaagttgcttaccacgaaaagtacccaactatctaccatttgagaaagaagttggttgactctaccgataaggctgatttgagattgatctatttggctttggcccacatgattaagttcagaggtcatttcttgatcgagggtgatttgaatccagataactccgatgttgacaagttgttcatccaattggtccaaacttacaaccagttgttcgaagaaaatccaatcaatgcctctggtgttgatgctaaggctattttgtctgctagactgtctaagtctagaaggttggaaaacttgattgctcaattgccaggtgaaaagaagaatggtttgttcggtaatttgatcgccttgtctttgggtttgactccaaatttcaagtccaacttcgatttggctgaagatgctaagttgcaattgtctaaggatacctacgatgatgacttggataatttgttggcccaaatcggtgatcaatacgctgatttgtttttggctgctaagaacttgtccgatgccattttgttgtccgatatcttgagagttaacaccgaaattactaaggctccattgtctgcctctatgatcaaaagatacgatgaacaccaccaagacttgactttgttgaaagctttggtcagacaacagttgccagaaaagtacaaagaaatcttcttcgaccagtccaaaaatggttacgctggttatattgatggtggtgcttctcaagaagagttctacaagttcattaagcccatcttggaaaagatggatggtactgaagaactgttggtcaagttgaacagagaagatttgttgagaaagcagagaaccttcgataacggttctattccacatcaaatccacttgggtgaattgcatgctattttgagaaggcaagaggatttctacccattcttgaaggataacagagaaaagatcgagaagatcctgaccttcagaattccatattatgttggtccattggccagaggtaattctagatttgcttggatgactaggaagtccgaagaaactattactccatggaacttcgaagaggttgttgataagggtgcttctgctcaatccttcattgaaagaatgactaacttcgacaagaacctgccaaacgaaaaggttttgccaaaacactctttgctgtacgaatacttcaccgtctacaacgaattgactaaggttaagtacgtcaccgaaggtatgagaaaaccagcttttttgtctggtgaacaaaagaaggctatcgtcgatttgttgttcaagactaacagaaaggttaccgtcaagcaattgaaagaggactacttcaagaaaatcgagtgcttcgattccgttgaaatttccggtgttgaagatagattcaacgcttccttaggtacttaccatgacctgttgaaaatcatcaaggacaaggatttcttggacaacgaagaaaacgaggatatcttggaggatatcgttttgactttgaccttgttcgaggatagggaaatgatcgaagaaaggttgaaaacctacgctcacttgtttgatgataaggtcatgaagcagttgaagagaagaaggtatactggttggggtagattgtctaggaaattgattaacggtatcagggacaagcaatccggtaagactattttggactttttgaagtctgatggcttcgccaatagaaacttcatgcaattgatccacgatgacagcttgaccttcaaagaagatattcaaaaggcccaagtttccggtcaaggtgattctttacatgaacatattgctaacttggctggttccccagctattaagaaaggtattttacaaaccgttaaggtggtcgacgaattggtaaaagttatgggtagacataagccagagaacatcgttattgaaatggctagagaaaatcagactacccaaaagggtcaaaagaactccagagaaaggatgaagagaattgaagagggtatcaaagaattgggctcccagattttgaaagaacacccagttgaaaacacccaattgcagaacgaaaagctgtacttgtactacttgcagaatggtagagatatgtacgtcgaccaagaattggatatcaacagattgtccgattacgatgtcgatcatatcgttccacagtcttttttgaaggatgactccatcgataacaaggtcttgactagatccgataagaacagaggtaagtctgataacgttccatctgaagaggtcgtcaagaagatgaagaattattggagacagttgctgaacgccaagttgattactcaaagaaagttcgacaatttgaccaaggctgaaagaggtggtttgtctgaattggacaaagcaggtttcattaagaggcaattggttgaaactaggcaaatcaccaaacacgttgcccaaattttggattccagaatgaataccaagtacgacgaaaacgataagttgatcagggaagttaaggtcatcacgttgaagtctaagttggtttccgatttcagaaaggacttccaattctacaaggtcagggaaatcaacaactaccatcatgctcatgatgcttacttgaatgctgttgttggtactgccttgattaagaagtatccaaagttggaatccgagttcgtttacggtgattacaaggtttacgacgtcagaaagatgattgccaagtccgaacaagaaattggtaaggctactgccaagtactttttctactccaacatcatgaatttcttcaagaccgaaatcactttggccaacggtgaaattagaaaaaggccattgattgagactaacggtgagactggtgaaatagtttgggataagggtagagatttcgctaccgttagaaaagttttgtccatgccacaagttaacatcgtcaaaaagaccgaagttcaaactggtggtttctccaaagaatccatcttgccaaaaagaaactccgacaaattgatcgccagaaagaaagattgggacccaaaaaagtatggcggttttgattctccaactgttgcttactctgttttggttgttgccaaagtcgaaaagggtaagagtaagaagttgaagtcagtcaaagagttgttgggtatcacgatcatggaaaggtcatctttcgaaaagaatcctatcgactttttggaagccaagggttacaaagaagtcaaaaaggacctgattatcaagctgccaaagtactctttgttcgaattggaaaacggtcgtaagagaatgttggcttctgctggtgaactacaaaaaggtaatgaattggctctgccctctaagtacgttaacttcttgtacttggcttctcactacgaaaagttgaaaggttctccagaagataacgagcaaaagcagttgtttgtggaacaacataagcactacttggacgaaatcatcgaacagatctctgaattctccaagagggttattttggctgatgccaatttggataaggtcttgtctgcttacaacaagcacagagataagccaattagagaacaagccgaaaacatcattcacctgttcactttgactaatttgggtgctccagctgcttttaagtacttcgatacaaccatcgacagaaagagatacacctctaccaaagaagttttggacgctaccttgatccatcaatctattactggtctgtacgaaaccagaatcgacttgtctcaattaggtggtgattaa

SEQ ID NO: 25 - DNA, 20 bp, synthetic construct
  misc_feature 1..20: note = SpCas9 Ade2 Spacer Sequence
  source 1..20: mol_type = other DNA
attgggacgtatgattgttg

SEQ ID NO: 26 - DNA, 76 bp, synthetic construct
  misc_feature 1..76: note = SpCas9 sgRNA Sequence
  source 1..76: mol_type = other DNA
gttttagagctagaaatagcaagttaaaataaggctagtccgttatcaacttgaaaaagtggcaccgagtcggtgc

SEQ ID NO: 27 - DNA, 8667 bp, synthetic construct
  misc_feature 1..8667: note = CRISPR/SpCas9 vector system
  source 1..8667: mol_type = other DNA
agcttgcaaattaaagccttcgagcgtcccaaaaccttctcaagcaaggttttcagtataatgttacatgcgtacacgcgtctgtacagaaaaaaaagaaaaatttgaaatataaataacgttcttaatactaacataactataaaaaaataaatagggacctagacttcaggttgtctaactccttccttttcggttagagcggatgtggggggagggcgtgaatgtaagcgtgacataactaattacatgatatcgacaaaggaaaagggggacggatctccgaggcctcggacccgtcgggccgcgtcggacgtgtcagtcctgctcctcgcaattgttagaaaaactcatcgagcatcaaatgaaactgcaatttattcatatcaggattatcaataccatatttttgaaaaagccgtttctgtaatgaaggagaaaactcaccgaggcagttccataggatggcaagatcctggtatcggtctgcgattccgactcgtccaacatcaatacaacctattaatttcccctcgtcaaaaataaggttatcaagtgagaaatcaccatgagtgacgactgaatccggtgagaatggcaaaagcttatgcatttctttccagacttgttcaacaggccagccattacgctcgtcatcaaaatcactcgcatcaaccaaaccgttattcattcgtgattgcgcctgagcgaggcgaaatacgcgatcgctgttaaaaggacaattacaaacaggaatcgaatgcaaccggcgcaggaacactgccagcgcatcaacaatattttcacctgaatcaggatattcttctaatacctggaatgctgttttgccggggatcgcagtggtgagtaaccatgcatcatcaggagtacggataaaatgcttgatggtcggaagaggcataaattccgtcagccagtttagtctgaccatctcatctgtaacatcattggcaacgctacctttgccatgtttcagaaacaactctggcgcatcgggcttcccatacaatcgatagattgtcgcacctgattgcccgacattatcgcgagcccatttatacccatataaatcagcatccatgttggaatttaatcgcggcctcgaaacgtgagtcttttccttacccatggtttagttcctcaccttgtcgtattatactatgccgatatactatgccgatgattaattgtcaacaccgcccttagattagattgctatgctttctttctaatgagcaagaagtaaaaaaagttgtaatagaacaagaaaaatgaaactgaaacttgagaaattgaagaccgtttattaacttaaatatcaatgggaggtcatcgaaagagaaaaaaatcaaaaaaaaaaattttcaagaaaaagaaacgtgataaaaatttttattgcctttttcgacgaagaaaaagaaacgaggcggtctcttttttcttttccaaacctttagtacgggtaattaacgacaccctagaggaagaaagaggggaaatttagtatgctgtgcttgggtgttttgaagtggtacggcgatgcgcggagtccgagaaaatctggaagagtaaaaaaggagtagaaacattttgaagctatggtgtgtgggggatccgcacaaacgaaggtctcactgatcgcttgcctgtaacttacacgcgcctcgtatcttttaatgatggaataatttgggaatttactctgtgtttatttatttttatgttttgtatttggattttagaaagtaaataaagaaggtagaagagttacggaatgaagaaaaaaaaataaacaaaggtttaaaaaatttcaacaaaaagcgtactttacatatatatttattagacaagaaaagcagattaaatagatatacattcgattaacgataagtaaaatgtaaaatcacaggattttcgtgtgtggtcttctacacagacaagatgaaacaattcggcattaatacctgagagcaggaagagcaagataaaaggtagtatttgttggcgatccccctagagtcttttacatcttcggaaaacaaaaactattttttctttaatttctttttttactttctatttttaatttatatatttatattaaaaaatttaaattataattatttttatagcacgtgatgaaaaggacccatcgataagctggtaccgagctcggatcccggtctgcatctgcggatcctctttgaaaagataatgtatgattatgctttcactcatatttatacagaaacttgatgttttctttcgagtatatacaaggtgattacatgtacgtttgaagtacaactctagattttgtagtgccctcttgggctagcggtaaaggtgcgcattttttcacaccctacaatgttctgttcaaaagattttggtcaaacgctgtagaagtgaaagttggtgcgcatgtttcggcgttcgaaacttctccgcagtgaaagataaatgatccgagacgagtctcggaagctcaaacgtctcatttttttgttttttatgtctcctgcaggtttaaagattacggatatttaacttacttagaataatgccatttttttgagttataataatcctacgttagtgtgagcgggatttaaactgtgaggaccttaatacattcagacacttctgcggtatcaccctacttattcccttcgagattatatctaggaacccatcaggttggtggaagattacccgttctaagacttttcagcttcctctattgatgttacacctggacaccccttttctggcatccagtttttaatcttcagtggcatgtgagattctccgaaattaattaaagcaatcacacaattctctcggataccacctcggttgaaactgacaggtggtttgttacgcatgctaatgcaaaggagcctatatacctttggctcggctgctgtaacagggaatataaagggcagcataatttaggagtttagtgaacttgcaacatttactattttcccttcttacgtaaatatttttctttttaattctaaatcaatctttttcaattttttgtttgtattcttttcttgcttaaatctataactacaaaaaacacatacataaactaaaaatggctcccaaaaagaaaaggaaggtgatggacaagaagtactccatcggtttggatattggtacaaattctgttggttgggccgttattactgatgagtacaaagttccatccaagaagttcaaggttttgggtaacactgataggcactccatcaaaaagaatttgattggtgccttgttgttcgactctggtgaaactgctgaagctactagattgaaaagaaccgctagaagaagatacaccagaagaaagaacagaatctgctacttgcaagagatcttctctaacgaaatggccaaggttgatgattcattcttccacagattggaagagtccttcttggttgaagaggataagaaacacgaaagacatccaatcttcggtaacatcgttgatgaagttgcttaccacgaaaagtacccaactatctaccatttgagaaagaagttggttgactctaccgataaggctgatttgagattgatctatttggctttggcccacatgattaagttcagaggtcatttcttgatcgagggtgatttgaatccagataactccgatgttgacaagttgttcatccaattggtccaaacttacaaccagttgttcgaagaaaatccaatcaatgcctctggtgttgatgctaaggctattttgtctgctagactgtctaagtctagaaggttggaaaacttgattgctcaattgccaggtgaaaagaagaatggtttgttcggtaatttgatcgccttgtctttgggtttgactccaaatttcaagtccaacttcgatttggctgaagatgctaagttgcaattgtctaaggatacctacgatgatgacttggataatttgttggcccaaatcggtgatcaatacgctgatttgtttttggctgctaagaacttgtccgatgccattttgttgtccgatatcttgagagttaacaccgaaattactaaggctccattgtctgcctctatgatcaaaagatacgatgaacaccaccaagacttgactttgttgaaagctttggtcagacaacagttgccagaaaagtacaaagaaatcttcttcgaccagtccaaaaatggttacgctggttatattgatggtggtgcttctcaagaagagttctacaagttcattaagcccatcttggaaaagatggatggtactgaagaactgttggtcaagttgaacagagaagatttgttgagaaagcagagaaccttcgataacggttctattccacatcaaatccacttgggtgaattgcatgctattttgagaaggcaagaggatttctacccattcttgaaggataacagagaaaagatcgagaagatcctgaccttcagaattccatattatgttggtccattggccagaggtaattctagatttgcttggatgactaggaagtccgaagaaactattactccatggaacttcgaagaggttgttgataagggtgcttctgctcaatccttcattgaaagaatgactaacttcgacaagaacctgccaaacgaaaaggttttgccaaaacactctttgctgtacgaatacttcaccgtctacaacgaattgactaaggttaagtacgtcaccgaaggtatgagaaaaccagcttttttgtctggtgaacaaaagaaggctatcgtcgatttgttgttcaagactaacagaaaggttaccgtcaagcaattgaaagaggactacttcaagaaaatcgagtgcttcgattccgttgaaatttccggtgttgaagatagattcaacgcttccttaggtacttaccatgacctgttgaaaatcatcaaggacaaggatttcttggacaacgaagaaaacgaggatatcttggaggatatcgttttgactttgaccttgttcgaggatagggaaatgatcgaagaaaggttgaaaacctacgctcacttgtttgatgataaggtcatgaagcagttgaagagaagaaggtatactggttggggtagattgtctaggaaattgattaacggtatcagggacaagcaatccggtaagactattttggactttttgaagtctgatggcttcgccaatagaaacttcatgcaattgatccacgatgacagcttgaccttcaaagaagatattcaaaaggcccaagtttccggtcaaggtgattctttacatgaacatattgctaacttggctggttccccagctattaagaaaggtattttacaaaccgttaaggtggtcgacgaattggtaaaagttatgggtagacataagccagagaacatcgttattgaaatggctagagaaaatcagactacccaaaagggtcaaaagaactccagagaaaggatgaagagaattgaagagggtatcaaagaattgggctcccagattttgaaagaacacccagttgaaaacacccaattgcagaacgaaaagctgtacttgtactacttgcagaatggtagagatatgtacgtcgaccaagaattggatatcaacagattgtccgattacgatgtcgatcatatcgttccacagtcttttttgaaggatgactccatcgataacaaggtcttgactagatccgataagaacagaggtaagtctgataacgttccatctgaagaggtcgtcaagaagatgaagaattattggagacagttgctgaacgccaagttgattactcaaagaaagttcgacaatttgaccaaggctgaaagaggtggtttgtctgaattggacaaagcaggtttcattaagaggcaattggttgaaactaggcaaatcaccaaacacgttgcccaaattttggattccagaatgaataccaagtacgacgaaaacgataagttgatcagggaagttaaggtcatcacgttgaagtctaagttggtttccgatttcagaaaggacttccaattctacaaggtcagggaaatcaacaactaccatcatgctcatgatgcttacttgaatgctgttgttggtactgccttgattaagaagtatccaaagttggaatccgagttcgtttacggtgattacaaggtttacgacgtcagaaagatgattgccaagtccgaacaagaaattggtaaggctactgccaagtactttttctactccaacatcatgaatttcttcaagaccgaaatcactttggccaacggtgaaattagaaaaaggccattgattgagactaacggtgagactggtgaaatagtttgggataagggtagagatttcgctaccgttagaaaagttttgtccatgccacaagttaacatcgtcaaaaagaccgaagttcaaactggtggtttctccaaagaatccatcttgccaaaaagaaactccgacaaattgatcgccagaaagaaagattgggacccaaaaaagtatggcggttttgattctccaactgttgcttactctgttttggttgttgccaaagtcgaaaagggtaagagtaagaagttgaagtcagtcaaagagttgttgggtatcacgatcatggaaaggtcatctttcgaaaagaatcctatcgactttttggaagccaagggttacaaagaagtcaaaaaggacctgattatcaagctgccaaagtactctttgttcgaattggaaaacggtcgtaagagaatgttggcttctgctggtgaactacaaaaaggtaatgaattggctctgccctctaagtacgttaacttcttgtacttggcttctcactacgaaaagttgaaaggttctccagaagataacgagcaaaagcagttgtttgtggaacaacataagcactacttggacgaaatcatcgaacagatctctgaattctccaagagggttattttggctgatgccaatttggataaggtcttgtctgcttacaacaagcacagagataagccaattagagaacaagccgaaaacatcattcacctgttcactttgactaatttgggtgctccagctgcttttaagtacttcgatacaaccatcgacagaaagagatacacctctaccaaagaagttttggacgctaccttgatccatcaatctattactggtctgtacgaaaccagaatcgacttgtctcaattaggtggtgattaagcggccgcaatgccggcgcaatgattgaatagtcaaagattttttttttttaattttttttttttaattttttttttttttcatagaactttttatttaaataaatcacgtctatatatgtatcagtataacgtaaaaaaaaaaacaccgtcagttaaacaaaacataaataaaaaaaaaaagaagtgtcaaatcaagtgtcaaatggccctgcattaatgaatcggccaacgcgcggggagaggcggtttgcgtattgggcgctcttccgcttcctcgctcactgactcgctgcgctcggtcgttcggctgcggcgagcggtatcagctcactcaaaggcggtaatacggttatccacagaatcaggggataacgcaggaaagaacatgtgagcaaaaggccagcaaaaggccaggaaccgtaaaaaggccgcgttgctggcgtttttccataggctccgcccccctgacgagcatcacaaaaatcgacgctcaagtcagaggtggcgaaacccgacaggactataaagataccaggcgtttccccctggaagctccctcgtgcgctctcctgttccgaccctgccgcttaccggatacctgtccgcctttctcccttcgggaagcgtggcgctttctcatagctcacgctgtaggtatctcagttcggtgtaggtcgttcgctccaagctgggctgtgtgcacgaaccccccgttcagcccgaccgctgcgccttatccggtaactatcgtcttgagtccaacccggtaagacacgacttatcgccactggcagcagccactggtaacaggattagcagagcgaggtatgtaggcggtgctacagagttcttgaagtggtggcctaactacggctacactagaagaacagtatttggtatctgcgctctgctgaagccagttaccttcggaaaaagagttggtagctcttgatccggcaaacaaaccaccgctggtagcggtggtttttttgtttgcaagcagcagattacgcgcagaaaaaaaggatctcaagaagatcctttgatcttttctacggggtctgacgctcagtggaacgaaaactcacgttaagggattttggtcatgagattatcaaaaaggatcttcacctagatccttttaaattaaaaatgaagttttaaatcaatctaaagtatatatgagtaaacttggtctgacagttaccaatgcttaatcagtgaggcacctatctcagcgatctgtctatttcgttcatccatagttgcctgactccccgtcgtgtagataactacgatacgggagggcttaccatctggccccagtgctgcaatgataccgcgagacccacgctcaccggctccagatttatcagcaataaaccagccagccggaagggc

SEQ ID NO: 28 - DNA, 832 bp, synthetic construct
  misc_feature 1..832: note = Ade2 HDR-template for SpCas9
  source 1..832: mol_type = other DNA
tctttacaacgaagttacctcttccatcgtatgccaaagtcctcgacttcaagacgaatggaaaacccaaatctcttccaacattcaatagggacgtctcactggcttgttccacaggaacactttgggtaactgctataccatttttgattaaatgctctttttgaatatatttgtcttgtatcaatctgattgtttctggagaagggtaaatttttaatttgggatgttttacttgaagattctttagtgtaggaacatcaacatgctcaatctcaatcgttagcacatcacatttttcagctagtttttcgatatcaagaggattggaaaaggagccattaacgtggtcattggagttgcttatttgtttggcaggagaattttcagcatctagtattaccgtcttaatgttgagcctgtttgctgtccccctcctaatataccaactgttctagaatccatacttgattgttttgtccgattttcttgtttttcttgattgttatagtaggatgtacttagaagagagatccaacgattttacgcaccaatttatacatgaaatgctccataatattgtccatttagttcttaataaaaggtcagcaagagtcaatcacttagtattacccggttcgtagccatgcaacaagagtcatttgtcagcatagctgtaataatcaatcatgacgtaagaaatgtatcataattaaaagttgttaaagatgtcagtgttatgttggtgttacaaaattctcggcttctcactaatatttaatatctcttaaattttatctgtctttgattcttttaagaaaagttatgtatt

SEQ ID NO: 29 - protein, 1231 aa, synthetic construct
  REGION 1..1231: note = AA Sequence of BEC10
MKSFENSCQISKTLRFGATLKEDKKKCKSHLELQEFVDISYKTLKSSATIAESLNEIELVKKCERCYSEIIKFHEAWGQIYCRTNQIAVYKDWYRQLARKARFDVGDQNSQLITLSSLSSKHNVYQGLKRSQHITNYWKDNIARQKSFLKDFSQQLKQYKRALENSDKAHTKPNLINFNKTFSILANLVNEIVIPLSNGAISFPNISKLEDGEESRHLIEFALNDYSDLVGSIGELKDAIATNGGYTPFAKVTLNHYTAEQKPHVFKNDIDAKIRELKLIELVEKLKNKTSKQIEEYFSKFDKFKIYDDRNISVIIRTQCFKYKPIPFLVKHELAKYIAEDEDAVLKVLDAIGATRSPAHDYAHNEDVFDLNHYPIKVAFDYAWEQLANGVYTTVTFPKEQCEKYLKDVFDCEVSKEPVFKFYADLLYIRKNLAVLEHKNNLPSNQEEFICKINNTFENIVLPYKIKEFETYKKDILAWINDGRGHEKYTDAKQQLGFIRGGLKGRIKAQKMFRKDKYGKIKSYYENPYTKLTNEFKQISSTYGKTFAELRDKFKEKNNITKITHFGIIIEDNNKDRYLLANGLQHEQINHVEAILGKLNTSSEFITYQVKSLTSKTLIKLIKNHTTKKGAISPYADFHTSKIHVDWTKIKKEWDNYKREQVLLQYVKDCLTDSTMAKNQNWAEFGWNFEKCNSYEDIEHEIDQKSYILQKHTISKQSIASLVEGGCLLLPIINQDITSQGRKDKNQFSKDWKQIFEGSKEFRLHPEFAVSYRTPIKDYPKDKRYGRLQFVCAFNCEIIPQNGEFINLKKQIENFNDEDAQKEAVEEFNKKVNHALLGKEYVVIGIDRGLKQLATLCVLDKRGKILGDFEIYKKEFVRAEKRSKNYWKHTLAETRHILDLSNLRVETTIEDNKVLVDQSLTLVKKNRDTPDEEATEENKQKIKLKQLSYIRKLQHKMQTNEQDVLDLINNEPSDEEFKKRIEGLISSFGEGQKYADLPINTMREMISDLQGVIARGNNQTEKNKIIELDAADNLKQGIVANMIGIVNYIFAKYSYKAYISLEDLSRAYGGAKSGYDGRYLPSTSQDEDVDFKEQQNQMLAGLGTYQFFEMQLLKKLQKIQSDNTVLRFVPAFRSADNYRNIIKLEETKYKSKPFGVVHFIDPKFTSKKCPVCSKTNVYRDKDDILVCKECGFRSDSQLKERENNIHYIHNGDDNGAYHIALKSVENLIQMK

SEQ ID NO: 30 - DNA, 3696 bp, synthetic construct
  misc_feature 1..3696: note = NT Sequence of BEC10 (Codon optimized for S. Cerevisiae)
  source 1..3696: mol_type = other DNA
atgaagtccttcgaaaactcctgccaaatttctaagactttgagattcggtgccactttgaaagaggataagaaaaagtgcaagtcccacttggaattgcaagaattcgttgacatttcctacaagaccttgaagtcatctgctaccattgctgaatccttgaacgaaatcgaattggtcaaaaagtgcgaaaggtgctactccgaaattatcaagttccatgaagcttggggtcaaatctactgtagaactaaccaaattgccgtctacaaggactggtatagacaattggctagaaaggccagattcgatgttggtgatcaaaactctcaactgatcaccttgtcatccttatcttctaagcacaacgtttaccagggtttgaagagatctcaacatattaccaactactggaaggacaacattgccagacaaaagtctttcctgaaggatttctctcaacaattgaagcagtacaagagagctttggaaaattctgataaggctcataccaagccaaacctgattaacttcaacaagaccttctccattttggccaacttggttaacgaaattgtcatcccattgtccaacggtgctatttcttttccaaacatctccaagttggaagatggtgaagaatccagacatttgattgaattcgctctgaacgattactccgatttggttggttctattggtgaattgaaggatgctattgctaccaatggtggttatactccatttgctaaggttaccttgaaccattacactgctgaacaaaagccacacgttttcaagaacgatattgatgccaagatccgtgagttgaagttgattgagttggtcgaaaagttgaagaacaagacgtccaagcaaatcgaagagtacttttccaagttcgacaagttcaagatctacgatgatagaaacatctccgttatcattagaacccaatgctttaagtacaagcccattccatttttggtcaagcacgaattggctaagtatatcgctgaagatgaagatgccgttttgaaggttttggatgcaattggtgctactagatctccagctcatgattacgctcataatgaagatgtttttgacttgaatcactacccaatcaaggttgcttttgattacgcatgggaacaattggctaacggtgtctacactactgttactttcccaaaagaacagtgcgagaagtacttgaaggatgtttttgattgcgaagtctccaaagaaccagtttttaagttctacgccgacctgttgtacatcagaaagaatttggctgttttggagcacaagaacaacctgccatctaatcaagaggaattcatctgcaagattaacaacaccttcgagaacatcgttctgccatacaagattaaagagttcgaaacctacaagaaggatatcttggcctggattaacgatggtagaggtcacgaaaagtacaccgatgctaaacaacagttgggttttattagaggtggtctgaaaggtagaatcaaggctcaaaagatgttcagaaaagacaagtacggtaagatcaagtcctactacgaaaacccatacactaagttgaccaacgaattcaagcaaatctcttctacctacggtaaaaccttcgctgaattgagagacaagttcaaagaaaagaacaacatcaccaagatcacccatttcggtattatcatcgaagataacaacaaagacagatacttgttggccaacggtttgcaacacgaacaaatcaaccatgtcgaagccattttgggtaagttgaacacctcatccgaattcatcacctaccaagttaagtctttgacctctaagaccctgatcaagctgattaagaatcataccaccaagaagggtgcaatttctccatatgctgatttccatacttctaagatccatgttgattggaccaagatcaagaaagaatgggacaactacaagagagaacaagtcttgttgcaatacgttaaggattgcttgaccgattctaccatggctaagaatcaaaattgggctgaatttggttggaacttcgagaagtgtaactcctacgaagatatcgaacacgaaatcgatcagaagtcttacatcttgcaaaagcataccatttccaagcaatctattgcttctttggttgaaggtggttgtttgttgttgccaattatcaaccaggacatcacctctcaaggtcgtaaggacaagaatcagttctccaaggattggaagcaaatcttcgaaggttccaaagaattcagattgcatccagaattcgccgtttcttacagaactccaattaaggactacccaaaggataaaagatacggtagattgcaattcgtttgcgcttttaactgcgaaatcatcccacaaaatggtgagttcatcaacttgaagaagcagatcgagaacttcaacgacgaagatgctcaaaaagaagccgtcgaagagttcaacaaaaaggttaaccatgccttgttgggtaaagaatacgttgttattggtatcgacagaggcttgaagcaattagctactttgtgtgttttggacaagaggggtaagattttgggtgactttgaaatctacaaaaaagagttcgtcagagccgaaaagagatctaagaattactggaagcacaccttggctgaaaccagacatatcttggacttgtctaacttgagagttgaaactaccattgaggataataaggtgttggttgatcaatctttgacactggtcaagaagaacagagatactccagatgaagaagctaccgaagaaaacaagcagaagattaagttgaagcagctgtcctacattagaaagttgcaacacaagatgcagaccaatgaacaagatgtcttggacctgatcaacaacgaaccatctgatgaagaattcaaaaagaggatcgagggcttgatttcttcattcggtgaaggtcaaaagtacgctgatttgcctattaacaccatgagggaaatgatctctgacttgcaaggtgttattgccagaggaaacaatcagactgagaaaaacaagatcatcgaattggatgctgccgacaatttgaaacaaggtatcgttgctaacatgatcggtatcgttaactacattttcgccaagtactcctacaaggcctacatttctttagaagatttgtccagagcttacggtggtgcaaaatctggttatgatggtagatatttgccatccacctctcaagatgaggatgttgactttaaagaacagcagaatcaaatgttggctggcttgggtacttaccaattttttgaaatgcagctgctgaaaaagctgcagaagatccaatctgataacaccgttttgagatttgttccagcttttagatccgccgataactacagaaatatcatcaagttggaagagactaagtacaagtctaagccattcggtgttgttcatttcatcgatccaaagttcacatctaagaagtgtccagtttgctctaagactaacgtttacagagataaggatgacatcctggtctgtaaagaatgtggttttaggtccgactcacagttgaaagaaagggaaaacaacatccactacatccacaatggtgatgataatggtgcttaccatattgccttgaagtccgtcgaaaacttgattcagatgaagtaa

SEQ ID NO: 31 - DNA, 8269 bp, synthetic construct
  misc_feature 1..8269: note = CRISPR/BEC10 vector system
  source 1..8269: mol_type = other DNA
agcttgcaaattaaagccttcgagcgtcccaaaaccttctcaagcaaggttttcagtataatgttacatgcgtacacgcgtctgtacagaaaaaaaagaaaaatttgaaatataaataacgttcttaatactaacataactataaaaaaataaatagggacctagacttcaggttgtctaactccttccttttcggttagagcggatgtggggggagggcgtgaatgtaagcgtgacataactaattacatgatatcgacaaaggaaaagggggacggatctccgaggcctcggacccgtcgggccgcgtcggacgtgtcagtcctgctcctcgcaattgttagaaaaactcatcgagcatcaaatgaaactgcaatttattcatatcaggattatcaataccatatttttgaaaaagccgtttctgtaatgaaggagaaaactcaccgaggcagttccataggatggcaagatcctggtatcggtctgcgattccgactcgtccaacatcaatacaacctattaatttcccctcgtcaaaaataaggttatcaagtgagaaatcaccatgagtgacgactgaatccggtgagaatggcaaaagcttatgcatttctttccagacttgttcaacaggccagccattacgctcgtcatcaaaatcactcgcatcaaccaaaccgttattcattcgtgattgcgcctgagcgaggcgaaatacgcgatcgctgttaaaaggacaattacaaacaggaatcgaatgcaaccggcgcaggaacactgccagcgcatcaacaatattttcacctgaatcaggatattcttctaatacctggaatgctgttttgccggggatcgcagtggtgagtaaccatgcatcatcaggagtacggataaaatgcttgatggtcggaagaggcataaattccgtcagccagtttagtctgaccatctcatctgtaacatcattggcaacgctacctttgccatgtttcagaaacaactctggcgcatcgggcttcccatacaatcgatagattgtcgcacctgattgcccgacattatcgcgagcccatttatacccatataaatcagcatccatgttggaatttaatcgcggcctcgaaacgtgagtcttttccttacccatggtttagttcctcaccttgtcgtattatactatgccgatatactatgccgatgattaattgtcaacaccgcccttagattagattgctatgctttctttctaatgagcaagaagtaaaaaaagttgtaatagaacaagaaaaatgaaactgaaacttgagaaattgaagaccgtttattaacttaaatatcaatgggaggtcatcgaaagagaaaaaaatcaaaaaaaaaaattttcaagaaaaagaaacgtgataaaaatttttattgcctttttcgacgaagaaaaagaaacgaggcggtctcttttttcttttccaaacctttagtacgggtaattaacgacaccctagaggaagaaagaggggaaatttagtatgctgtgcttgggtgttttgaagtggtacggcgatgcgcggagtccgagaaaatctggaagagtaaaaaaggagtagaaacattttgaagctatggtgtgtgggggatccgcacaaacgaaggtctcactgatcgcttgcctgtaacttacacgcgcctcgtatcttttaatgatggaataatttgggaatttactctgtgtttatttatttttatgttttgtatttggattttagaaagtaaataaagaaggtagaagagttacggaatgaagaaaaaaaaataaacaaaggtttaaaaaatttcaacaaaaagcgtactttacatatatatttattagacaagaaaagcagattaaatagatatacattcgattaacgataagtaaaatgtaaaatcacaggattttcgtgtgtggtcttctacacagacaagatgaaacaattcggcattaatacctgagagcaggaagagcaagataaaaggtagtatttgttggcgatccccctagagtcttttacatcttcggaaaacaaaaactattttttctttaatttctttttttactttctatttttaatttatatatttatattaaaaaatttaaattataattatttttatagcacgtgatgaaaaggacccatcgataagctggtaccgagctcggatcccggtctgcatctgcggatcctctttgaaaagataatgtatgattatgctttcactcatatttatacagaaacttgatgttttctttcgagtatatacaaggtgattacatgtacgtttgaagtacaactctagattttgtagtgccctcttgggctagcggtaaaggtgcgcattttttcacaccctacaatgttctgttcaaaagattttggtcaaacgctgtagaagtgaaagttggtgcgcatgtttcggcgttcgaaacttctccgcagtgaaagataaatgatcgaatttctactgttgtagatgtgtaggaacatcaacatgctcaatttttttgttttttatgtctcctgcaggtttaaagattacggatatttaacttacttagaataatgccatttttttgagttataataatcctacgttagtgtgagcgggatttaaactgtgaggaccttaatacattcagacacttctgcggtatcaccctacttattcccttcgagattatatctaggaacccatcaggttggtggaagattacccgttctaagacttttcagcttcctctattgatgttacacctggacaccccttttctggcatccagtttttaatcttcagtggcatgtgagattctccgaaattaattaaagcaatcacacaatgctctcggataccacctcggttgaaactgacaggtggtttgttacgcatgctaatgcaaaggagcctatatacctttggctcggctgctgtaacagggaatataaagggcagcataatttaggagtttagtgaacttgcaacatttactattttcccttcttacgtaaatatttttctttttaattctaaatcaatctttttcaattttttgtttgtattcttttcttgcttaaatctataactacaaaaaacacatacataaactaaaaatggctcccaaaaagaaaaggaaggtgatgaagtccttcgaaaactcctgccaaatttctaagactttgagattcggtgccactttgaaagaggataagaaaaagtgcaagtcccacttggaattgcaagaattcgttgacatttcctacaagaccttgaagtcatctgctaccattgctgaatccttgaacgaaatcgaattggtcaaaaagtgcgaaaggtgctactccgaaattatcaagttccatgaagcttggggtcaaatctactgtagaactaaccaaattgccgtctacaaggactggtatagacaattggctagaaaggccagattcgatgttggtgatcaaaactctcaactgatcaccttgtcatccttatcttctaagcacaacgtttaccagggtttgaagagatctcaacatattaccaactactggaaggacaacattgccagacaaaagtctttcctgaaggatttctctcaacaattgaagcagtacaagagagctttggaaaattctgataaggctcataccaagccaaacctgattaacttcaacaagaccttctccattttggccaacttggttaacgaaattgtcatcccattgtccaacggtgctatttcttttccaaacatctccaagttggaagatggtgaagaatccagacatttgattgaattcgctctgaacgattactccgatttggttggttctattggtgaattgaaggatgctattgctaccaatggtggttatactccatttgctaaggttaccttgaaccattacactgctgaacaaaagccacacgttttcaagaacgatattgatgccaagatccgtgagttgaagttgattgagttggtcgaaaagttgaagaacaagacgtccaagcaaatcgaagagtacttttccaagttcgacaagttcaagatctacgatgatagaaacatctccgttatcattagaacccaatgctttaagtacaagcccattccatttttggtcaagcacgaattggctaagtatatcgctgaagatgaagatgccgttttgaaggttttggatgcaattggtgctactagatctccagctcatgattacgctcataatgaagatgtttttgacttgaatcactacccaatcaaggttgcttttgattacgcatgggaacaattggctaacggtgtctacactactgttactttcccaaaagaacagtgcgagaagtacttgaaggatgtttttgattgcgaagtctccaaagaaccagtttttaagttctacgccgacctgttgtacatcagaaagaatttggctgttttggagcacaagaacaacctgccatctaatcaagaggaattcatctgcaagattaacaacaccttcgagaacatcgttctgccatacaagattaaagagttcgaaacctacaagaaggatatcttggcctggattaacgatggtagaggtcacgaaaagtacaccgatgctaaacaacagttgggttttattagaggtggtctgaaaggtagaatcaaggctcaaaagatgttcagaaaagacaagtacggtaagatcaagtcctactacgaaaacccatacactaagttgaccaacgaattcaagcaaatctcttctacctacggtaaaaccttcgctgaattgagagacaagttcaaagaaaagaacaacatcaccaagatcacccatttcggtattatcatcgaagataacaacaaagacagatacttgttggccaacggtttgcaacacgaacaaatcaaccatgtcgaagccattttgggtaagttgaacacctcatccgaattcatcacctaccaagttaagtctttgacctctaagaccctgatcaagctgattaagaatcataccaccaagaagggtgcaatttctccatatgctgatttccatacttctaagatccatgttgattggaccaagatcaagaaagaatgggacaactacaagagagaacaagtcttgttgcaatacgttaaggattgcttgaccgattctaccatggctaagaatcaaaattgggctgaatttggttggaacttcgagaagtgtaactcctacgaagatatcgaacacgaaatcgatcagaagtcttacatcttgcaaaagcataccatttccaagcaatctattgcttctttggttgaaggtggttgtttgttgttgccaattatcaaccaggacatcacctctcaaggtcgtaaggacaagaatcagttctccaaggattggaagcaaatcttcgaaggttccaaagaattcagattgcatccagaattcgccgtttcttacagaactccaattaaggactacccaaaggataaaagatacggtagattgcaattcgtttgcgcttttaactgcgaaatcatcccacaaaatggtgagttcatcaacttgaagaagcagatcgagaacttcaacgacgaagatgctcaaaaagaagccgtcgaagagttcaacaaaaaggttaaccatgccttgttgggtaaagaatacgttgttattggtatcgacagaggcttgaagcaattagctactttgtgtgttttggacaagaggggtaagattttgggtgactttgaaatctacaaaaaagagttcgtcagagccgaaaagagatctaagaattactggaagcacaccttggctgaaaccagacatatcttggacttgtctaacttgagagttgaaactaccattgaggataataaggtgttggttgatcaatctttgacactggtcaagaagaacagagatactccagatgaagaagctaccgaagaaaacaagcagaagattaagttgaagcagctgtcctacattagaaagttgcaacacaagatgcagaccaatgaacaagatgtcttggacctgatcaacaacgaaccatctgatgaagaattcaaaaagaggatcgagggcttgatttcttcattcggtgaaggtcaaaagtacgctgatttgcctattaacaccatgagggaaatgatctctgacttgcaaggtgttattgccagaggaaacaatcagactgagaaaaacaagatcatcgaattggatgctgccgacaatttgaaacaaggtatcgttgctaacatgatcggtatcgttaactacattttcgccaagtactcctacaaggcctacatttctttagaagatttgtccagagcttacggtggtgcaaaatctggttatgatggtagatatttgccatccacctctcaagatgaggatgttgactttaaagaacagcagaatcaaatgttggctggcttgggtacttaccaattttttgaaatgcagctgctgaaaaagctgcagaagatccaatctgataacaccgttttgagatttgttccagcttttagatccgccgataactacagaaatatcatcaagttggaagagactaagtacaagtctaagccattcggtgttgttcatttcatcgatccaaagttcacatctaagaagtgtccagtttgctctaagactaacgtttacagagataaggatgacatcctggtctgtaaagaatgtggttttaggtccgactcacagttgaaagaaagggaaaacaacatccactacatccacaatggtgatgataatggtgcttaccatattgccttgaagtccgtcgaaaacttgattcagatgaagtaagcggccgcaatgccggcgcaatgattgaatagtcaaagattttttttttttaattttttttttttaattttttttttttttcatagaactttttatttaaataaatcacgtctatatatgtatcagtataacgtaaaaaaaaaaacaccgtcagttaaacaaaacataaataaaaaaaaaaagaagtgtcaaatcaagtgtcaaatggccctgcattaatgaatcggccaacgcgcggggagaggcggtttgcgtattgggcgctcttccgcttcctcgctcactgactcgctgcgctcggtcgttcggctgcggcgagcggtatcagctcactcaaaggcggtaatacggttatccacagaatcaggggataacgcaggaaagaacatgtgagcaaaaggccagcaaaaggccaggaaccgtaaaaaggccgcgttgctggcgtttttccataggctccgcccccctgacgagcatcacaaaaatcgacgctcaagtcagaggtggcgaaacccgacaggactataaagataccaggcgtttccccctggaagctccctcgtgcgctctcctgttccgaccctgccgcttaccggatacctgtccgcctttctcccttcgggaagcgtggcgctttctcatagctcacgctgtaggtatctcagttcggtgtaggtcgttcgctccaagctgggctgtgtgcacgaaccccccgttcagcccgaccgctgcgccttatccggtaactatcgtcttgagtccaacccggtaagacacgacttatcgccactggcagcagccactggtaacaggattagcagagcgaggtatgtaggcggtgctacagagttcttgaagtggtggcctaactacggctacactagaagaacagtatttggtatctgcgctctgctgaagccagttaccttcggaaaaagagttggtagctcttgatccggcaaacaaaccaccgctggtagcggtggtttttttgtttgcaagcagcagattacgcgcagaaaaaaaggatctcaagaagatcctttgatcttttctacggggtctgacgctcagtggaacgaaaactcacgttaagggattttggtcatgagattatcaaaaaggatcttcacctagatccttttaaattaaaaatgaagttttaaatcaatctaaagtatatatgagtaaacttggtctgacagttaccaatgcttaatcagtgaggcacctatctcagcgatctgtctatttcgttcatccatagttgcctgactccccgtcgtgtagataactacgatacgggagggcttaccatctggccccagtgctgcaatgataccgcgagacccacgctcaccggctccagatttatcagcaataaaccagccagccggaagggc

SEQ ID NO: 32 - DNA, 8272 bp, synthetic construct
  misc_feature 1..8272: note = CRISPR/SuCms1 vector system
  source 1..8272: mol_type = other DNA
agcttgcaaattaaagccttcgagcgtcccaaaaccttctcaagcaaggttttcagtataatgttacatgcgtacacgcgtctgtacagaaaaaaaagaaaaatttgaaatataaataacgttcttaatactaacataactataaaaaaataaatagggacctagacttcaggttgtctaactccttccttttcggttagagcggatgtggggggagggcgtgaatgtaagcgtgacataactaattacatgatatcgacaaaggaaaagggggacggatctccgaggcctcggacccgtcgggccgcgtcggacgtgtcagtcctgctcctcgcaattgttagaaaaactcatcgagcatcaaatgaaactgcaatttattcatatcaggattatcaataccatatttttgaaaaagccgtttctgtaatgaaggagaaaactcaccgaggcagttccataggatggcaagatcctggtatcggtctgcgattccgactcgtccaacatcaatacaacctattaatttcccctcgtcaaaaataaggttatcaagtgagaaatcaccatgagtgacgactgaatccggtgagaatggcaaaagcttatgcatttctttccagacttgttcaacaggccagccattacgctcgtcatcaaaatcactcgcatcaaccaaaccgttattcattcgtgattgcgcctgagcgaggcgaaatacgcgatcgctgttaaaaggacaattacaaacaggaatcgaatgcaaccggcgcaggaacactgccagcgcatcaacaatattttcacctgaatcaggatattcttctaatacctggaatgctgttttgccggggatcgcagtggtgagtaaccatgcatcatcaggagtacggataaaatgcttgatggtcggaagaggcataaattccgtcagccagtttagtctgaccatctcatctgtaacatcattggcaacgctacctttgccatgtttcagaaacaactctggcgcatcgggcttcccatacaatcgatagattgtcgcacctgattgcccgacattatcgcgagcccatttatacccatataaatcagcatccatgttggaatttaatcgcggcctcgaaacgtgagtcttttccttacccatggtttagttcctcaccttgtcgtattatactatgccgatatactatgccgatgattaattgtcaacaccgcccttagattagattgctatgctttctttctaatgagcaagaagtaaaaaaagttgtaatagaacaagaaaaatgaaactgaaacttgagaaattgaagaccgtttattaacttaaatatcaatgggaggtcatcgaaagagaaaaaaatcaaaaaaaaaaattttcaagaaaaagaaacgtgataaaaatttttattgcctttttcgacgaagaaaaagaaacgaggcggtctcttttttcttttccaaacctttagtacgggtaattaacgacaccctagaggaagaaagaggggaaatttagtatgctgtgcttgggtgttttgaagtggtacggcgatgcgcggagtccgagaaaatctggaagagtaaaaaaggagtagaaacattttgaagctatggtgtgtgggggatccgcacaaacgaaggtctcactgatcgcttgcctgtaacttacacgcgcctcgtatcttttaatgatggaataatttgggaatttactctgtgtttatttatttttatgttttgtatttggattttagaaagtaaataaagaaggtagaagagttacggaatgaagaaaaaaaaataaacaaaggtttaaaaaatttcaacaaaaagcgtactttacatatatatttattagacaagaaaagcagattaaatagatatacattcgattaacgataagtaaaatgtaaaatcacaggattttcgtgtgtggtcttctacacagacaagatgaaacaattcggcattaatacctgagagcaggaagagcaagataaaaggtagtatttgttggcgatccccctagagtcttttacatcttcggaaaacaaaaactattttttctttaatttctttttttactttctatttttaatttatatatttatattaaaaaatttaaattataattatttttatagcacgtgatgaaaaggacccatcgataagctggtaccgagctcggatcccggtctgcatctgcggatcctctttgaaaagataatgtatgattatgctttcactcatatttatacagaaacttgatgttttctttcgagtatatacaaggtgattacatgtacgtttgaagtacaactctagattttgtagtgccctcttgggctagcggtaaaggtgcgcattttttcacaccctacaatgttctgttcaaaagattttggtcaaacgctgtagaagtgaaagttggtgcgcatgtttcggcgttcgaaacttctccgcagtgaaagataaatgatcgaatttctactgttgtagatgtgtaggaacatcaacatgctcaatttttttgttttttatgtctcctgcaggtttaaagattacggatatttaacttacttagaataatgccatttttttgagttataataatcctacgttagtgtgagcgggatttaaactgtgaggaccttaatacattcagacacttctgcggtatcaccctacttattcccttcgagattatatctaggaacccatcaggttggtggaagattacccgttctaagacttttcagcttcctctattgatgttacacctggacaccccttttctggcatccagtttttaatcttcagtggcatgtgagattctccgaaattaattaaagcaatcacacaattctctcggataccacctcggttgaaactgacaggtggtttgttacgcatgctaatgcaaaggagcctatatacctttggctcggctgctgtaacagggaatataaagggcagcataatttaggagtttagtgaacttgcaacatttactattttcccttcttacgtaaatatttttctttttaattctaaatcaatctttttcaattttttgtttgtattcttttcttgcttaaatctataactacaaaaaacacatacataaactaaaaatggctcccaaaaagaaaaggaaggtgatgttgcatgccttcaccaatcaataccaattgtctaagactttgagattcggtgccactttgaaagaagatgagaaaaagtgcaagtcccacgaagaattgaagggtttcgttgatatctcctacgagaacatgaagtcctctgctactattgctgaatccttgaacgaaaacgagttggtcaaaaagtgtgaaaggtgctactctgaaatcgtcaagtttcataatgcctgggagaagatctactacagaactgatcaaattgccgtctacaaggacttctacagacagttgtctagaaaggctagatttgatgctggtaagcaaaactcccaattgattactttggcttctttgtgcggtatgtaccaaggtgctaaattgtccagatatatcaccaattactggaaggacaacatcaccagacaaaagtctttcttgaaggatttctcccaacaattgcatcagtacactagagctttggaaaagtctgataaggctcataccaagccaaacttgatcaacttcaacaagaccttcatggttttggccaacttggttaacgaaatcgttatcccattgtccaacggtgctatttctttcccaaacatctctaagttggaagatggtgaagaatcccacttgattgaattcgctttgaacgactactctcagttgtctgaattgatcggtgaattgaaagatgctattgctaccaatggtggttacactccatttgctaaggttaccttgaatcattacaccgctgaacaaaagccacacgttttcaagaatgatatcgatgccaagatccgtgagttgaaattgataggtttggtcgaaaccttgaagggcaaatcctctgaacaaatcgaagagtactttagcaacctggataagttctctacctacaacgacagaaatcaatccgttatcgttagaacccaatgcttcaagtataagcccattccatttttggtcaagcaccaattggcaaagtacatctctgaacctaatggttgggatgaagatgctgttgcaaaagttttggatgcagttggtgctattagatctccagctcatgattacgctaacaatcaagaaggttttgacttgaatcactacccaatcaaggttgcttttgattacgcatgggaacaattggctaactccttgtacactactgttactttcccacaagaaatgtgcgagaagtacttgaattctatctacggttgcgaagtctccaaagaaccagtttttaagttctacgccgacctgttgtacatcagaaagaatttggctgttttggagcacaagaacaacctgccatctaatcaagaggaattcatctgcaagattaacaacaccttcgagaacatcgttctgccatacaagatttctcaattcgaaacctacaagaaggatatcttggcctggattaacgatggtcatgatcacaaaaagtacaccgatgctaaacaacagttgggttttattagaggtggtctgaaaggtagaatcaaggctgaagaagtttcccaaaaagacaagtacggtaagatcaagtcctactacgaaaacccatacactaagttgaccaacgaattcaagcaaatctcttctacctacggtaaaaccttcgctgaattgagagacaagttcaaagaaaagaacgagatcaccaagatcacccatttcggtattatcatcgaagataagaacagggacagatacttgttggcctcagaattgaaacacgaacaaatcaaccatgtctccaccatcttgaacaagttggataagtcatccgaattcatcacctaccaagttaagtctttgacctctaagaccctgatcaagctgattaagaatcataccaccaagaagggtgcaatttctccatatgctgatttccatacttctaagaccggctttaacaaaaacgagatcgaaaagaactgggacaactacaagagagaacaagtcttggttgaatacgttaaggattgcttgaccgattctaccatggctaagaatcaaaattgggctgaatttggttggaacttcgagaagtgtaactcctacgaagatatcgaacacgaaatcgatcagaagtcttacttgttgcaatccgacaccatttccaagcaatctattgcttctttggttgaaggtggttgtttgttgttgccaattatcaaccaggacatcacctctaaagaacgtaaggacaagaatcagttctccaaggattggaaccatatcttcgaaggttccaaagaattcagattgcatccagaattcgccgtttcttacagaactccaattgaaggttacccagtccaaaaaagatacggtagattgcaattcgtttgcgcttttaacgctcatatcgttccacaaaatggtgagttcatcaacttgaagaagcagatcgagaacttcaacgacgaagatgttcaaaagagaaacgttaccgagttcaacaaaaaggttaaccatgccttgtccgacaaagaatacgttgttattggtatcgacagaggcttgaagcaattagctactttgtgtgttttggacaagaggggtaagattttgggtgactttgaaatctacaaaaaagagttcgtcagagccgaaaagagatctgaatctcattgggaacatactcaagctgaaaccagacatatcttggacttgtctaacttgagagttgaaactaccattgagggcaaaaaggtgttggttgatcaatctttgacactggtcaagaagaacagagatactccagatgaagaagctaccgaagaaaacaagcagaagattaagttgaagcagctgtcctacattagaaagttgcaacacaagatgcagaccaatgaacaagatgtcttggacctgatcaacaacgaaccatctgatgaagaattcaaaaagaggatcgagggcttgatttcttcattcggtgaaggtcaaaagtacgctgatttgcctattaacaccatgagggaaatgatctctgacttgcaaggtgttattgccagaggaaacaatcagactgagaaaaacaagatcatcgaattggatgctgccgacaatttgaaacaaggtatcgttgctaacatgatcggtatcgttaactacattttcgccaagtactcctacaaggcctacatttctttagaagatttgtccagagcttacggtggtgcaaaatctggttatgatggtagatatttgccatccacctctcaagatgaggatgttgactttaaagaacagcagaatcaaatgttggctggcttgggtacttaccaattttttgaaatgcagctgctgaaaaagctgcagaagatccaatctgataacaccgttttgagatttgttccagcttttagatccgccgataactacagaaatatcttgagattggaagagactaagtacaagtctaagccattcggtgttgttcatttcatcgatccaaagttcacatctaagaagtgtccagtttgctctaagactaacgtttacagagataaggatgacatcctggtctgtaaagaatgtggttttaggtccgactcacagttgaaagaaagggaaaacaacatccactacatccacaatggtgatgataatggtgcttaccatattgccttgaagtccgtcgaaaacttgattcagatgaagtaagcggccgcaatgccggcgcaatgattgaatagtcaaagattttttttttttaattttttttttttaattttttttttttttcatagaactttttatttaaataaatcacgtctatatatgtatcagtataacgtaaaaaaaaaaacaccgtcagttaaacaaaacataaataaaaaaaaaaagaagtgtcaaatcaagtgtcaaatggccctgcattaatgaatcggccaacgcgcggggagaggcggtttgcgtattgggcgctcttccgcttcctcgctcactgactcgctgcgctcggtcgttcggctgcggcgagcggtatcagctcactcaaaggcggtaatacggttatccacagaatcaggggataacgcaggaaagaacatgtgagcaaaaggccagcaaaaggccaggaaccgtaaaaaggccgcgttgctggcgtttttccataggctccgcccccctgacgagcatcacaaaaatcgacgctcaagtcagaggtggcgaaacccgacaggactataaagataccaggcgtttccccctggaagctccctcgtgcgctctcctgttccgaccctgccgcttaccggatacctgtccgcctttctcccttcgggaagcgtggcgctttctcatagctcacgctgtaggtatctcagttcggtgtaggtcgttcgctccaagctgggctgtgtgcacgaaccccccgttcagcccgaccgctgcgccttatccggtaactatcgtcttgagtccaacccggtaagacacgacttatcgccactggcagcagccactggtaacaggattagcagagcgaggtatgtaggcggtgctacagagttcttgaagtggtggcctaactacggctacactagaagaacagtatttggtatctgcgctctgctgaagccagttaccttcggaaaaagagttggtagctcttgatccggcaaacaaaccaccgctggtagcggtggtttttttgtttgcaagcagcagattacgcgcagaaaaaaaggatctcaagaagatcctttgatcttttctacggggtctgacgctcagtggaacgaaaactcacgttaagggattttggtcatgagattatcaaaaaggatcttcacctagatccttttaaattaaaaatgaagttttaaatcaatctaaagtatatatgagtaaacttggtctgacagttaccaatgcttaatcagtgaggcacctatctcagcgatctgtctatttcgttcatccatagttgcctgactccccgtcgtgtagataactacgatacgggagggcttaccatctggccccagtgctgcaatgataccgcgagacccacgctcaccggctccagatttatcagcaataaaccagccagccggaagggc

SEQ ID NO: 33 - DNA, 8404 bp, synthetic construct
  misc_feature 1..8404: note = CRISPR/SeqID63 vector system
  source 1..8404: mol_type = other DNA
agcttgcaaattaaagccttcgagcgtcccaaaaccttctcaagcaaggttttcagtataatgttacatgcgtacacgcgtctgtacagaaaaaaaagaaaaatttgaaatataaataacgttcttaatactaacataactataaaaaaataaatagggacctagacttcaggttgtctaactccttccttttcggttagagcggatgtggggggagggcgtgaatgtaagcgtgacataactaattacatgatatcgacaaaggaaaagggggacggatctccgaggcctcggacccgtcgggccgcgtcggacgtgtcagtcctgctcctcgcaattgttagaaaaactcatcgagcatcaaatgaaactgcaatttattcatatcaggattatcaataccatatttttgaaaaagccgtttctgtaatgaaggagaaaactcaccgaggcagttccataggatggcaagatcctggtatcggtctgcgattccgactcgtccaacatcaatacaacctattaatttcccctcgtcaaaaataaggttatcaagtgagaaatcaccatgagtgacgactgaatccggtgagaatggcaaaagcttatgcatttctttccagacttgttcaacaggccagccattacgctcgtcatcaaaatcactcgcatcaaccaaaccgttattcattcgtgattgcgcctgagcgaggcgaaatacgcgatcgctgttaaaaggacaattacaaacaggaatcgaatgcaaccggcgcaggaacactgccagcgcatcaacaatattttcacctgaatcaggatattcttctaatacctggaatgctgttttgccggggatcgcagtggtgagtaaccatgcatcatcaggagtacggataaaatgcttgatggtcggaagaggcataaattccgtcagccagtttagtctgaccatctcatctgtaacatcattggcaacgctacctttgccatgtttcagaaacaactctggcgcatcgggcttcccatacaatcgatagattgtcgcacctgattgcccgacattatcgcgagcccatttatacccatataaatcagcatccatgttggaatttaatcgcggcctcgaaacgtgagtcttttccttacccatggtttagttcctcaccttgtcgtattatactatgccgatatactatgccgatgattaattgtcaacaccgcccttagattagattgctatgctttctttctaatgagcaagaagtaaaaaaagttgtaatagaacaagaaaaatgaaactgaaacttgagaaattgaagaccgtttattaacttaaatatcaatgggaggtcatcgaaagagaaaaaaatcaaaaaaaaaaattttcaagaaaaagaaacgtgataaaaatttttattgcctttttcgacgaagaaaaagaaacgaggcggtctcttttttcttttccaaacctttagtacgggtaattaacgacaccctagaggaagaaagaggggaaatttagtatgctgtgcttgggtgttttgaagtggtacggcgatgcgcggagtccgagaaaatctggaagagtaaaaaaggagtagaaacattttgaagctatggtgtgtgggggatccgcacaaacgaaggtctcactgatcgcttgcctgtaacttacacgcgcctcgtatcttttaatgatggaataatttgggaatttactctgtgtttatttatttttatgttttgtatttggattttagaaagtaaataaagaaggtagaagagttacggaatgaagaaaaaaaaataaacaaaggtttaaaaaatttcaacaaaaagcgtactttacatatatatttattagacaagaaaagcagattaaatagatatacattcgattaacgataagtaaaatgtaaaatcacaggattttcgtgtgtggtcttctacacagacaagatgaaacaattcggcattaatacctgagagcaggaagagcaagataaaaggtagtatttgttggcgatccccctagagtcttttacatcttcggaaaacaaaaactattttttctttaatttctttttttactttctatttttaatttatatatttatattaaaaaatttaaattataattatttttatagcacgtgatgaaaaggacccatcgataagctggtaccgagctcggatcccggtctgcatctgcggatcctctttgaaaagataatgtatgattatgctttcactcatatttatacagaaacttgatgttttctttcgagtatatacaaggtgattacatgtacgtttgaagtacaactctagattttgtagtgccctcttgggctagcggtaaaggtgcgcattttttcacaccctacaatgttctgttcaaaagattttggtcaaacgctgtagaagtgaaagttggtgcgcatgtttcggcgttcgaaacttctccgcagtgaaagataaatgatcgaatttctactgttgtagatgtgtaggaacatcaacatgctcaatttttttgttttttatgtctcctgcaggtttaaagattacggatatttaacttacttagaataatgccatttttttgagttataataatcctacgttagtgtgagcgggatttaaactgtgaggaccttaatacattcagacacttctgcggtatcaccctacttattcccttcgagattatatctaggaacccatcaggttggtggaagattacccgttctaagacttttcagcttcctctattgatgttacacctggacaccccttttctggcatccagtttttaatcttcagtggcatgtgagattctccgaaattaattaaagcaatcacacaattctctcggataccacctcggttgaaactgacaggtggtttgttacgcatgctaatgcaaaggagcctatatacctttggctcggctgctgtaacagggaatataaagggcagcataatttaggagtttagtgaacttgcaacatttactattttcccttcttacgtaaatatttttctttttaattctaaatcaatctttttcaattttttgtttgtattcttttcttgcttaaatctataactacaaaaaacacatacataaactaaaaatggctcccaaaaagaaaaggaaggtgatgaagtccttcgaaaactcctgccaaatttctaagactttgagattcggtgccactttgaaagaggataagaaaaagtgcaagtcccacgaagaattgcaagaattcgttgacatttcctacaagaccatgaagtcatctgctaccattgctgaatccttgaacgaaatcgaattggtcaaaaagtgcgaaaggtgctactccgaaattatcaagttccatgaagcttggggtcaaatctactgtagaactgatcaaattgccgtctacaaggacttctatagacaattggctagaaaggccagattcgatgttggtgatcaaaactctcaactgatcaccttgtcatccttatcttctaagcacaacgtttaccagggtttgaagagatctcaacatattaccaactactggaaggacaacattgccagacaaaagtctttcctgaaggatttctctcaacaattgcaccagtacaagagagctttggaaaattctgataaggctcataccaagccaaacctgattaacttcaacaagaccttctccattttggccaacttggttaacgaaattgtcatcccattgtccaacggtgctatttcttttccaaacatctccaagttggaagatggtgaagaatccagacatttgattgaattcgctctgaacgattactccgatttggttggttctattggtgaattgaaggatgctattgctaccaatggtggttatactccatttgctaaggttaccttgaaccattacactgctgaacaaaagccacacgttttcaagaacgatattgatgccaagatccgtgagttgaagttgattgagttggtcgaaaagttgaagaacaagacgtccaagcaaatcgaagagtacttttccaagttcgacaagttcaagatctacgatgatagaaaccagtccgttatcattagaacccaatgctttaagtacaagcccattccatttttggtcaagcacgaattggctaagtatatcgctgaagatgaagatgccgttttgaaggttttggatgcaattggtgctactagatctccagctcatgattacgctcataacgaagatgttttcgacttgaaacactacccaatcaaggttgcttttgattacgcatgggaacaattggcaaatggtgtttacactactgtctcattccctgaagaaaagtgcagagaatacttgaatgctatctacggttgcgaagttaccaaagaaccagtttttaagttctacgccgacctgttgtacatcagaaagaatttggctgttttggagcacaagaacaacttgccatctaatccagaagaattcatctgcaagattgagaacactttcgagaagatcgttctgccctacaagatcaaagaattcgaaacttacaagaaggccatcttgacctggattaacgatggtagaggtcacgaaaagtacaccgattctaaaagagaattgggtttgatcagaggtggtttgaaaggtagaattggtgcccaaaagatgttccgtaaaaacaagaaaggtgagttgatcccctactacgaaaatccatacactaagttgactaacgagttcaagaacatctcctcctcttacggtaaaactttcgctgaattgagggataagttcaaagagaagtctgagattaccaagatcacccatttcggtatcatcatcgaagataacaacaaggacagatacttgttggctaatggcttgcaacatgataacaccgatcaatctaacacccaagttgaagccattttgggtaaattgaacacctctttggaattcactacctaccaagttaagtccttgacctccaagattctgatcaagttgattaagaaccataccacctctccaaatgctaaatctccatacgctgatttccatacctctaagattcatgttgattggacgaagatcaagaaagaatgggatacctacaagtccaaccactctttgttgcaatatgttaaggactgtttgaccaactctaccatggctaagaatcaaaattgggctgaattcggttgggacttagaatcttgtaattcctacgaagccatcgaacacgagattgatcaaaagtcctacatcttgcaaaagcacaccatttctaaggcctccattaagtctttggttgaaaacggttgtctgttgttgccaatcgtcaatcaagatattacctctcaaggtcgtaaggacaagaatcaattttctaaggactggaagcaaatcttcgaggactctaaagagtacagattgcatcctgaatttgccgtttcttacagaaccccaatcaaagattatccaaaggataagaggtacggcagattgcaattcatttgtgctttcaactgcgaaatcatcccacaaaatggtgagttcatcaacctgaagaagcagatcgaaaacttcaacgacgaagatatccaaaagaacaatgtcgccgaattcaacaacaaagttaacgaagctttgctgggcaaagaatacgttgttattggtatcgatagaggcttgaaacagttggctactttgtgtgttttaaacaagaggggtaagatcttgggtgacttcgagatctacaagaaagagtttgttagaaccgagaacaggtctaagaattactggaaacatactttggccgaaaccagacatatcctggatttgtctaatttgagagttgaaaccaccgttgaggataacaaagttttggtcgatcaatccttgacgttggtcaagaagaatagagatactccagacgaaaaagccaccgaagagaatagacaaaagatcaagctgaagcagctgtcctacattagaaagttgcaatacgctatgcagaccaacgaacaagctgttttagatctgttgaaggataactccgacgatgaggaattcaaaaaaagagttgaaggcgtcatttccccatttggtgaaggtcaagaatatgctgatttgcctattgataccatgagagccatgattcaagacttgcaaggtgttattgctaagggtaacaagcaaaccgagaagaacaaaatcattgaattggatgctgccgactctttgaaacaaggtgttgtagctaatatgatcggcgttgttaacttcatcttggccaaattcaattacgaggcctacgtttctttggaggatttgtcaagagcttacaatgttgctaagtctggttatgacggtagatacttaccatccacttctcaagatccagatatggacttcaaagaacaacagaatcaaatgctagctggtttgggtacttaccagttcttcgaaattcagctgttgaagaagttgcagaagatccaatccaacaacactgttttgagatttgtcccagcttttagatccgctgataactacagaaacatcatcaaactgaaccccaagtacgacaacactgaatatgttcataagccattcggtatcgttcacttcattgatcctaaggatacctcttctaagtgtccagtttgtggtaagactggtaaaaagaacgttgacagaaacgagaagaaaaacaacatcttgttgtgtaaggcttgcggttttagaacagtctgggaattgaaacaaccagagaacatcaaatctgagggttactgtttttccgaggacgaaattcaaaagaccattaagaacaatcaaaaacagatggaaatcaagaagctgtccgataagaacatccattacatccataacggtgatgataatggtgcttaccatattgccttgaagtctgtcgagaatttgaagcacaaagaataagcggccgcaatgccggcgcaatgattgaatagtcaaagattttttttttttaattttttttttttaattttttttttttttcatagaactttttatttaaataaatcacgtctatatatgtatcagtataacgtaaaaaaaaaaacaccgtcagttaaacaaaacataaataaaaaaaaaaagaagtgtcaaatcaagtgtcaaatggccctgcattaatgaatcggccaacgcgcggggagaggcggtttgcgtattgggcgctcttccgcttcctcgctcactgactcgctgcgctcggtcgttcggctgcggcgagcggtatcagctcactcaaaggcggtaatacggttatccacagaatcaggggataacgcaggaaagaacatgtgagcaaaaggccagcaaaaggccaggaaccgtaaaaaggccgcgttgctggcgtttttccataggctccgcccccctgacgagcatcacaaaaatcgacgctcaagtcagaggtggcgaaacccgacaggactataaagataccaggcgtttccccctggaagctccctcgtgcgctctcctgttccgaccctgccgcttaccggatacctgtccgcctttctcccttcgggaagcgtggcgctttctcatagctcacgctgtaggtatctcagttcggtgtaggtcgttcgctccaagctgggctgtgtgcacgaaccccccgttcagcccgaccgctgcgccttatccggtaactatcgtcttgagtccaacccggtaagacacgacttatcgccactggcagcagccactggtaacaggattagcagagcgaggtatgtaggcggtgctacagagttcttgaagtggtggcctaactacggctacactagaagaacagtatttggtatctgcgctctgctgaagccagttaccttcggaaaaagagttggtagctcttgatccggcaaacaaaccaccgctggtagcggtggtttttttgtttgcaagcagcagattacgcgcagaaaaaaaggatctcaagaagatcctttgatcttttctacggggtctgacgctcagtggaacgaaaactcacgttaagggattttggtcatgagattatcaaaaaggatcttcacctagatccttttaaattaaaaatgaagttttaaatcaatctaaagtatatatgagtaaacttggtctgacagttaccaatgcttaatcagtgaggcacctatctcagcgatctgtctatttcgttcatccatagttgcctgactccccgtcgtgtagataactacgatacgggagggcttaccatctggccccagtgctgcaatgataccgcgagacccacgctcaccggctccagatttatcagcaataaaccagccagccggaagggc

SEQ ID NO: 34 - DNA, 10407 bp, synthetic construct
  misc_feature 1..10407: note = CRISPR/BEC10_Coli vector system
  source 1..10407: mol_type = other DNA
ccatgcttatctccatgcggtagggtgccgcacggttgcggcaccatgcgcaatcagctgcaacttttcggcagcgcgacaacaattatgcgttgcgtaaaagtggcagtcaattacagattttctttaacctacgcaatgagctattgcggggggtgccgcaatgagctgttgcgtaccccccttttttaagttgttgatttttaagtctttcgcatttcgccctatatctagttctttggtgcccaaagaagggcacccctgcggggttcccccacgccttcggcgcggctccccctccggcaaaaagtggcccctccggggcttgttgatcgactgcgcggccttcggccttgcccaaggtggcgctgcccccttggaacccccgcactcgccgccgtgaggctcggggggcaggcgggcgggcttcgccttcgactgcccccactcgcataggcttgggtcgttccaggcgcgtcaaggccaagccgctgcgcggtcgctgcgcgagccttgacccgccttccacttggtgtccaaccggcaagcgaagcgcgcaggccgcaggccggaggcttttccccagagaaaattaaaaaaattgatggggcaaggccgcaggccgcgcagttggagccggtgggtatgtggtcgaaggctgggtagccggtgggcaatccctgtggtcaagctcgtgggcaggcgcagcctgtccatcagcttgtccagcagggttgtccacgggccgagcgaagcgagccagccggtggccgctcgcggccatcgtccacatatccacgggctggcaagggagcgcagcgaccgcgcagggcgaagcccggagagcaagcccgtagggcgccgcagccgccgtaggcggtcacgactttgcgaagcaaagtctagtgagtatactcaagcattgagtggcccgccggaggcaccgccttgcgctgcccccgtcgagccggttggacaccaaaagggaggggcaggcatggcggcatacgcgatcatgcgatgcaagaagctggcgaaaatgggcaacgtggcggccagtctcaagcacgcctaccgcgagcgcgagacgcccaacgctgacgccagcaggacgccagagaacgagcactgggcggccagcagcaccgatgaagcgatgggccgactgcgcgagttgctgccagagaagcggcgcaaggacgctgtgttggcggtcgagtacgtcatgacggccagcccggaatggtggaagtcggccagccaagaacagcaggcggcgttcttcgagaaggcgcacaagtggctggcggacaagtacggggcggatcgcatcgtgacggccagcatccaccgtgacgaaaccagcccgcacatgaccgcgttcgtggtgccgctgacgcaggacggcaggctgtcggccaaggagttcatcggcaacaaagcgcagatgacccgcgaccagaccacgtttgcggccgctgtggccgatctagggctgcaacggggcatcgagggcagcaaggcacgtcacacgcgcattcaggcgttctacgaggccctggagcggccaccagtgggccacgtcaccatcagcccgcaagcggtcgagccacgcgcctatgcaccgcagggattggccgaaaagctgggaatctcaaagcgcgttgagacgccggaagccgtggccgaccggctgacaaaagcggttcggcaggggtatgagcctgccctacaggccgccgcaggagcgcgtgagatgcgcaagaaggccgatcaagcccaagagacggcccgagaccttcgggagcgcctgaagcccgttctggacgccctggggccgttgaatcgggatatgcaggccaaggccgccgcgatcatcaaggccgtgggcgaaaagctgctgacggaacagcgggaagtccagcgccagaaacaggcccagcgccagcaggaacgcgggcgcgcacatttccccgaaaagtgccacctgaaccccagagtcccgctcagaagaactcgtcaagaaggcgatagaaggcgatgcgctgcgaatcgggagcggcgataccgtaaagcacgaggaagcggtcagcccattcgccgccaagctcttcagcaatatcacgggtagccaacgctatgtcctgatagcggtccgccacacccagccggccacagtcgatgaatccagaaaagcggccattttccaccatgatattcggcaagcaggcatcgccatgggtcacgacgagatcctcgccgtcgggcatccgcgccttgagcctggcgaacagttcggctggcgcgagcccctgatgctcttcgtccagatcatcctgatcgacaagaccggcttccatccgagtacgtgctcgctcgatgcgatgtttcgcttggtggtcgaatgggcaggtagccggatcaagcgtatgcagccgccgcattgcatcagccatgatggatactttctcggcaggagcaaggtgagatgacaggagatcctgccccggcacttcgcccaatagcagccagtcccttcccgcttcagtgacaacgtcgagcacagctgcgcaaggaacgcccgtcgtggccagccacgatagccgcgctgcctcgtcttggagttcattcagggcaccggacaggtcggtcttgacaaaaagaaccgggcgcccctgcgctgacagccggaacacggcggcatcagagcagccgattgtctgttgtgcccagtcatagccgaatagcctctccacccaagcggccggagaacctgcgtgcaatccatcttgttcaatcatgcgaaacgatcctcatcctgtctcttgatcagatcttgatcccctgcgccatcagatccttggcggcaagaaagccatccagtttactttgcagggcttcccaaccttaccagagggcgccccagctggcaattccggttcgcttgctgtccataaaaccgcccagtctagctatcgccatgtaagcccactgcaagctacctgctttctctttgcgcttgcgttttcccttgtccagatagcccagtagctgacattcatccggggtcagcaccgtttctgcggactggctttctacgtgttccgcttcctttagcagcccttgcgccctgagtgcttgcggcagcgtgaagctagcataaaacgaaaggcccagtctttcgactgagcctttcgttttatttgatgcctggcagttccctactctcgcatggggagaccccacactaccatcggcgctacggcgtttcacttctgagttcggcatggggtcaggtgggaccaccgcgctactgccgccaggcaaaaaaaaaagtcccggttgagtacatcgcaggatctacaacagtagaaattcgacctcattctattagactctcgtttggattgcaactggtctattttcctcttttgtttgatagaaaatcataaaaggatttgcagactacgggcctaaagaactaaaaaatctatctgtttcttttcattctctgtattttttatagtttctgttgcatgggctgcataatgtgcctgtcaaatggacgaagcagggattctgcaaaccctatgctactccgtcaagccgtcaattgtctgattcgttaccaattatgacaacttgacggctacatcattcactttttcttcacaaccggcacggaactcgctcgggctggccccggtgcattttttaaatacccgcgagaaatagagttgatcgtcaaaaccaacattgcgaccgacggtggcgataggcatccgggtggtgctcaaaagcagcttcgcctggctgatacgttggtcctcgcgccagcttaagacgctaatccctaactgctggcggaaaagatgtgacagacgcgacggcgacaagcaaacatgctgtgcgacgctggcgatatcaaaattgctgtctgccaggtgatcgctgatgtactgacaagcctcgcgtacccgattatccatcggtggatggagcgactcgttaatcgcttccatgcgccgcagtaacaattgctcaagcagatttatcgccagcagctccgaatagcgcccttccccttgcccggcgttaatgatttgcccaaacaggtcgctgaaatgcggctggtgcgcttcatccgggcgaaagaaccccgtattggcaaatattgacggccagttaagccattcatgccagtaggcgcgcggacgaaagtaaacccactggtgataccattcgcgagcctccggatgacgaccgtagtgatgaatctctcctggcgggaacagcaaaatatcacccggtcggcaaacaaattctcgtccctgatttttcaccaccccctgaccgcgaatggtgagattgagaatataacctttcattcccagcggtcggtcgataaaaaaatcgagataaccgttggcctcaatcggcgttaaacccgccaccagatgggcattaaacgagtatcccggcagcaggggatcattttgcgcttcagccatacttttcatactcccgccattcagagaagaaaccaattgtccatattgcatcagacattgccgtcactgcgtcttttactggctcttctcgctaaccaaaccggtaaccccgcttattaaaagcattctgtaacaaagcgggaccaaagccatgacaaaaacgcgtaacaaaagtgtctataatcacggcagaaaagtccacattgattatttgcacggcgtcacactttgctatgccatagcatttttatccataagattagcggatcctacctgacgctttttatcgcaactctctactgtttctccatacccgttttttggtaccgggccccccctcgagtttattttaggaggcaaaaatgaaaagctttgaaaacagctgccagattagcaaaaccctgcgttttggtgcaaccctgaaagaggataaaaagaaatgtaaaagccacctggaactgcaagaatttgtggatattagctacaagaccctgaaaagcagcgcaaccattgcagaaagcctgaatgaaattgagctggtgaaaaaatgcgaacgctgctatagcgaaatcatcaaatttcatgaagcctggggtcagatttattgtcgtaccaatcagattgccgtgtacaaagattggtatcgtcagctggcacgtaaagcacgttttgatgttggtgatcagaatagccagctgattaccctgagcagcctgagtagcaaacataatgtttatcagggtctgaaacgcagccagcatattaccaattattggaaagataacattgcccgtcagaaaagcttcctgaaagattttagccagcagctgaaacagtataaacgtgcactggaaaatagcgataaagcacataccaaaccgaacctgatcaacttcaataaaacctttagcattctggccaacctggtgaacgaaattgttattccgctgagcaatggtgcaattagctttccgaatatcagcaaactggaagatggtgaagaaagccgtcatctgattgaatttgccctgaatgattatagcgatctggttggtagcattggcgaactgaaagatgcaattgccaccaatggtggttataccccgtttgcaaaagttaccctgaaccattataccgcagaacagaaaccgcatgtgttcaaaaatgatatcgatgccaaaatccgtgagctgaaactgattgaactggttgagaaactgaaaaacaaaaccagcaagcagatcgaagagtacttcagcaaattcgacaagttcaaaatctatgatgatcgcaacatcagcgtgattattcgtacccagtgctttaaatacaaaccgattccgtttctggtgaaacatgaactggccaaatatatcgccgaagatgaagatgcagttctgaaagttctggatgccattggtgcgacccgtagtccggcacatgattatgcacataatgaagatgtgttcgatctgaaccactatccgattaaagtggcatttgattatgcctgggaacagctggcaaatggtgtgtataccaccgtgacctttccgaaagaacagtgtgaaaaatatctgaaggatgtgtttgattgcgaggttagcaaagaaccggtgtttaaattctatgccgatctgctgtatatccgcaaaaatctggccgttctggaacataaaaacaatctgccgagcaaccaagaagagttcatttgcaaaatcaacaacaccttcgaaaacatcgtgctgccgtataaaatcaaagagttcgaaacctacaaaaaagacatcctggcctggattaatgatggtcgtggtcatgagaaatataccgatgcaaaacagcagctgggttttattcgtggtggtctgaaaggtcgtattaaagcccagaaaatgttccgcaaagataagtacggtaagatcaaaagctattatgagaacccgtataccaaactgaccaacgaatttaagcagatcagcagcacctatggcaaaacctttgccgaactgcgtgataagtttaaagagaagaacaacatcaccaaaatcacccactttggcatcatcatcgaggataataacaaagatcgttatctgctggccaatggtctgcagcatgagcagattaatcatgttgaagcaattctgggcaaactgaataccagcagcgaatttatcacctatcaggttaaaagcctgaccagtaaaaccctgattaagctgattaaaaaccataccaccaaaaagggtgcgattagcccgtatgcagattttcataccagcaaaattcatgtggactggacgaaaatcaaaaaagagtgggataactataagcgcgaacaggttctgctgcagtatgttaaagattgtctgaccgatagcaccatggccaaaaatcagaattgggcagaatttggctggaactttgaaaaatgcaacagctatgaagatatcgagcacgagattgaccagaaaagttatatcctgcagaaacacaccatctccaaacagagcattgcaagcctggttgaaggtggttgtctgctgctgccgattattaaccaggatattacctcacagggtcgcaaagacaaaaaccagtttagtaaagattggaagcagatctttgaaggcagcaaagaatttcgtctgcatccggaatttgcagttagctatcgtaccccgatcaaagattatccgaaagataaacgttatggtcgcctgcagtttgtttgtgcctttaactgtgaaatcattccgcagaatggcgaattcatcaatctgaaaaagcagattgagaacttcaacgatgaggatgcacagaaagaagccgttgaagaattcaacaaaaaagtgaatcatgccctgctgggcaaagaatatgttgtgattggtattgatcgtggcctgaaacaactggcaaccctgtgtgttctggataaacgtggtaaaatcctgggcgattttgagatctacaagaaagaattcgttcgtgccgaaaaacgcagcaaaaactattggaaacacacactggcagaaacccgtcatattctggatctgagcaatctgcgtgttgaaaccacaatcgaagataacaaagtgctggttgatcagagtctgaccctggttaaaaagaatcgtgatacaccggatgaagaagccaccgaagaaaataaacagaagatcaaactgaagcagctgagctatattcgtaaactgcagcataaaatgcagaccaatgaacaggatgttctggacctgattaataacgaaccgagcgacgaagaatttaagaaacgtattgaaggtctgattagcagctttggtgaaggtcagaaatatgcggatctgcctattaataccatgcgcgaaatgattagtgatctgcagggtgttattgcccgtggtaataatcagacagagaaaaacaagatcatcgaactggatgcagccgataatctgaaacagggtattgttgcaaacatgattggcatcgtgaactacatctttgccaaatacagctacaaagcctatatcagcctggaagatctgagccgtgcatatggtggtgcaaaaagcggttatgatggacgctatctgccgtcaaccagccaggacgaagatgtggattttaaagaacagcagaatcagatgctggcaggtctgggtacatatcagttttttgaaatgcagctgctgaagaagctgcagaaaattcagagcgataataccgttctgcgctttgttccggcatttcgtagcgcagataactatcgcaatattatcaagctggaagaaaccaaatacaaaagcaaaccgtttggcgtggtgcactttattgatccgaaatttacgagcaaaaaatgtccggtttgcagcaaaaccaatgtgtatcgtgataaagatgacattctggtgtgtaaagaatgcggttttcgtagtgatagtcagctgaaagaacgcgaaaacaacatccactatattcataatggtgatgacaacggtgcctatcatattgcactgaaaagcgtggaaaatctgatccagatgaaataatggtctagaggtcgaaattcaaattgtgagcggataacaatttgaattttctgtatgaggttttgctaaacaactttcaacagtttcagtggagtgagaatagaaaggaacaactaaaggaattgcgaataataattttttcacgttgaaaatctccaaaaaaaaaggctccaaaaggagcctttaattgtatcggtttatcagcttgctttcgaggtgaattttgaccctctagcgaaaatgcaagagcaaagacgaaaacatgccacacatgaggaataccgattctctcattaacatattcaggccagttatctgggcttaaaagcagaagtccaacccagataacgatcatatacatggttctctccagaggttcattactgaacactcgtccgagaataacgagtggatcccctccaattcgccctatagtgagtcgtattacgcgcgctcactggccgtcgttttacaacgtcgtgactgggaaaaccctggcgttacccaacttaatcgccttgcagcacatccccctttcgccagctggcgtaatagcgaagaggcccgcaccgatcgcccttcccaacagttgcgcagcctgaatggcgaatggaaattgtaagcgttaatattttgttaaaattcgcgttaaatttttgttaaatcagctcattttttaaccaataggccgactgcgatgagtggcagggcggggcgtaatttttttaaggcagttattggtgcccttaaacgcctggtgctacgcctgaataagtgataataagcggatgaatggcagaaattcgaaagcaaattcgacccggtcgtcggttcagggcagggtcgttaaatagccgcttatgtctattgctggtttaccggtttattgactaccggaagcagtgtgaccgtgtgcttctcaaatgcctgaggccagtttgctcaggctctccccgtggaggtaataattgacgatatgatcatttattctgcctcccagagcctgataaaaacggtgaatccgttagcgaggtgccgccggcttccattcaggtcgaggtggcccggctccatgcaccgcgacgcaacgcggggaggcagacaaggtatagggcggcgaggcggctacagccgatagtctggaacagcgcacttacgggttgctgcgcaacccaagtgctaccggcgcggcagcgtgacccgtgtcggcggctccaacggctcgccatcgtccagaaaacacggctcatcgggcatcggcaggcgctgctgcccgcgccgttcccattcctccgtttcggtcaaggctggcaggtctggttccatgcccggaatgccgggctggctgggcggctcctcgccggggccggtcggtagttgctgctcgcccggatacagggtcgggatgcggcgcaggtcgccatgccccaacagcgattcgtcctggtcgtcgtgatcaaccaccacggcggcactgaacaccgacaggcgcaactggtcgcggggctggccccacgccacgcggtcattgaccacgtaggccgacacggtgccggggccgttgagcttcacgacggagatccagcgctcggccaccaagtccttgactgcgtattggaccgtccgcaaagaacgtccgatgagcttggaaagtgtcttttggctgaccaccacggcgttctggtggcccatctgcgccacgaggtgatgcagcagcattgccgccgtgggtttcctcgcaataagcccggcccacgcctcatgcgctttgcgttccgtttgcacccagtgaccgggcttgttcttggcttgaatgccgatttctctggactgcgtgg

SEQ ID NO: 35 - DNA, 10410 bp, synthetic construct
  misc_feature 1..10410: note = CRISPR/SuCms1_Coli vector system
  source 1..10410: mol_type = other DNA
ccatgcttatctccatgcggtagggtgccgcacggttgcggcaccatgcgcaatcagctgcaacttttcggcagcgcgacaacaattatgcgttgcgtaaaagtggcagtcaattacagattttctttaacctacgcaatgagctattgcggggggtgccgcaatgagctgttgcgtaccccccttttttaagttgttgatttttaagtctttcgcatttcgccctatatctagttctttggtgcccaaagaagggcacccctgcggggttcccccacgccttcggcgcggctccccctccggcaaaaagtggcccctccggggcttgttgatcgactgcgcggccttcggccttgcccaaggtggcgctgcccccttggaacccccgcactcgccgccgtgaggctcggggggcaggcgggcgggcttcgccttcgactgcccccactcgcataggcttgggtcgttccaggcgcgtcaaggccaagccgctgcgcggtcgctgcgcgagccttgacccgccttccacttggtgtccaaccggcaagcgaagcgcgcaggccgcaggccggaggcttttccccagagaaaattaaaaaaattgatggggcaaggccgcaggccgcgcagttggagccggtgggtatgtggtcgaaggctgggtagccggtgggcaatccctgtggtcaagctcgtgggcaggcgcagcctgtccatcagcttgtccagcagggttgtccacgggccgagcgaagcgagccagccggtggccgctcgcggccatcgtccacatatccacgggctggcaagggagcgcagcgaccgcgcagggcgaagcccggagagcaagcccgtagggcgccgcagccgccgtaggcggtcacgactttgcgaagcaaagtctagtgagtatactcaagcattgagtggcccgccggaggcaccgccttgcgctgcccccgtcgagccggttggacaccaaaagggaggggcaggcatggcggcatacgcgatcatgcgatgcaagaagctggcgaaaatgggcaacgtggcggccagtctcaagcacgcctaccgcgagcgcgagacgcccaacgctgacgccagcaggacgccagagaacgagcactgggcggccagcagcaccgatgaagcgatgggccgactgcgcgagttgctgccagagaagcggcgcaaggacgctgtgttggcggtcgagtacgtcatgacggccagcccggaatggtggaagtcggccagccaagaacagcaggcggcgttcttcgagaaggcgcacaagtggctggcggacaagtacggggcggatcgcatcgtgacggccagcatccaccgtgacgaaaccagcccgcacatgaccgcgttcgtggtgccgctgacgcaggacggcaggctgtcggccaaggagttcatcggcaacaaagcgcagatgacccgcgaccagaccacgtttgcggccgctgtggccgatctagggctgcaacggggcatcgagggcagcaaggcacgtcacacgcgcattcaggcgttctacgaggccctggagcggccaccagtgggccacgtcaccatcagcccgcaagcggtcgagccacgcgcctatgcaccgcagggattggccgaaaagctgggaatctcaaagcgcgttgagacgccggaagccgtggccgaccggctgacaaaagcggttcggcaggggtatgagcctgccctacaggccgccgcaggagcgcgtgagatgcgcaagaaggccgatcaagcccaagagacggcccgagaccttcgggagcgcctgaagcccgttctggacgccctggggccgttgaatcgggatatgcaggccaaggccgccgcgatcatcaaggccgtgggcgaaaagctgctgacggaacagcgggaagtccagcgccagaaacaggcccagcgccagcaggaacgcgggcgcgcacatttccccgaaaagtgccacctgaaccccagagtcccgctcagaagaactcgtcaagaaggcgatagaaggcgatgcgctgcgaatcgggagcggcgataccgtaaagcacgaggaagcggtcagcccattcgccgccaagctcttcagcaatatcacgggtagccaacgctatgtcctgatagcggtccgccacacccagccggccacagtcgatgaatccagaaaagcggccattttccaccatgatattcggcaagcaggcatcgccatgggtcacgacgagatcctcgccgtcgggcatccgcgccttgagcctggcgaacagttcggctggcgcgagcccctgatgctcttcgtccagatcatcctgatcgacaagaccggcttccatccgagtacgtgctcgctcgatgcgatgtttcgcttggtggtcgaatgggcaggtagccggatcaagcgtatgcagccgccgcattgcatcagccatgatggatactttctcggcaggagcaaggtgagatgacaggagatcctgccccggcacttcgcccaatagcagccagtcccttcccgcttcagtgacaacgtcgagcacagctgcgcaaggaacgcccgtcgtggccagccacgatagccgcgctgcctcgtcttggagttcattcagggcaccggacaggtcggtcttgacaaaaagaaccgggcgcccctgcgctgacagccggaacacggcggcatcagagcagccgattgtctgttgtgcccagtcatagccgaatagcctctccacccaagcggccggagaacctgcgtgcaatccatcttgttcaatcatgcgaaacgatcctcatcctgtctcttgatcagatcttgatcccctgcgccatcagatccttggcggcaagaaagccatccagtttactttgcagggcttcccaaccttaccagagggcgccccagctggcaattccggttcgcttgctgtccataaaaccgcccagtctagctatcgccatgtaagcccactgcaagctacctgctttctctttgcgcttgcgttttcccttgtccagatagcccagtagctgacattcatccggggtcagcaccgtttctgcggactggctttctacgtgttccgcttcctttagcagcccttgcgccctgagtgcttgcggcagcgtgaagctagcataaaacgaaaggcccagtctttcgactgagcctttcgttttatttgatgcctggcagttccctactctcgcatggggagaccccacactaccatcggcgctacggcgtttcacttctgagttcggcatggggtcaggtgggaccaccgcgctactgccgccaggcaaaaaaaaaagtcccggttgagtacatcgcaggatctacaacagtagaaattcgacctcattctattagactctcgtttggattgcaactggtctattttcctcttttgtttgatagaaaatcataaaaggatttgcagactacgggcctaaagaactaaaaaatctatctgtttcttttcattctctgtattttttatagtttctgttgcatgggctgcataatgtgcctgtcaaatggacgaagcagggattctgcaaaccctatgctactccgtcaagccgtcaattgtctgattcgttaccaattatgacaacttgacggctacatcattcactttttcttcacaaccggcacggaactcgctcgggctggccccggtgcattttttaaatacccgcgagaaatagagttgatcgtcaaaaccaacattgcgaccgacggtggcgataggcatccgggtggtgctcaaaagcagcttcgcctggctgatacgttggtcctcgcgccagcttaagacgctaatccctaactgctggcggaaaagatgtgacagacgcgacggcgacaagcaaacatgctgtgcgacgctggcgatatcaaaattgctgtctgccaggtgatcgctgatgtactgacaagcctcgcgtacccgattatccatcggtggatggagcgactcgttaatcgcttccatgcgccgcagtaacaattgctcaagcagatttatcgccagcagctccgaatagcgcccttccccttgcccggcgttaatgatttgcccaaacaggtcgctgaaatgcggctggtgcgcttcatccgggcgaaagaaccccgtattggcaaatattgacggccagttaagccattcatgccagtaggcgcgcggacgaaagtaaacccactggtgataccattcgcgagcctccggatgacgaccgtagtgatgaatctctcctggcgggaacagcaaaatatcacccggtcggcaaacaaattctcgtccctgatttttcaccaccccctgaccgcgaatggtgagattgagaatataacctttcattcccagcggtcggtcgataaaaaaatcgagataaccgttggcctcaatcggcgttaaacccgccaccagatgggcattaaacgagtatcccggcagcaggggatcattttgcgcttcagccatacttttcatactcccgccattcagagaagaaaccaattgtccatattgcatcagacattgccgtcactgcgtcttttactggctcttctcgctaaccaaaccggtaaccccgcttattaaaagcattctgtaacaaagcgggaccaaagccatgacaaaaacgcgtaacaaaagtgtctataatcacggcagaaaagtccacattgattatttgcacggcgtcacactttgctatgccatagcatttttatccataagattagcggatcctacctgacgctttttatcgcaactctctactgtttctccatacccgttttttggtaccgggccccccctcgagtttattttaggaggcaaaaatgctgcatgcatttaccaatcagtatcagctgagcaaaaccctgcgttttggtgcaaccctgaaagaagatgagaaaaaatgcaaaagccacgaggaactgaaaggctttgttgatattagctatgaaaacatgaaaagcagcgcaaccattgcagaaagcctgaatgaaaatgagctggtgaaaaaatgtgaacgctgctatagcgagatcgtgaaattccataatgcctgggagaaaatctattatcgcaccgatcagattgccgtgtataaagatttttatcgtcagctgagtcgcaaagcacgttttgatgcaggtaaacagaatagccagctgattaccctggcaagcctgtgtggtatgtatcagggtgcaaaactgagccgttatattaccaattactggaaggataacatcacccgtcagaagagttttctgaaagattttagccagcagctgcatcagtatacccgtgcactggaaaaaagcgataaagcacataccaaaccgaacctgatcaacttcaataaaacctttatggtgctggccaatctggtgaacgaaattgttattccgctgagcaatggtgcaattagctttccgaatatcagcaaactggaagatggtgaagaaagccatctgattgaatttgccctgaacgattattcacagctgagcgaactgattggcgagctgaaagatgcaattgccaccaatggtggttataccccgtttgcaaaagttaccctgaatcattataccgcagaacagaaaccgcacgtgtttaaaaacgatatcgatgccaaaatccgcgaactgaaactgatcggtctggttgaaacactgaaaggtaaaagcagtgagcagatcgaagaatatttcagcaacctggataaattcagcacctataatgatcgtaaccagagcgttattgttcgtacccagtgctttaaatacaaaccgattccgtttctggtgaaacatcaactggccaaatatatcagcgaaccgaatggttgggatgaagatgcagttgcgaaagttctggatgccgttggtgccattcgtagtccggcacatgattatgcaaataaccaagaaggctttgatctgaaccactatccgattaaagtggcctttgattatgcgtgggaacagctggcaaatagcctgtataccaccgttacctttccgcaagaaatgtgcgaaaaatatctgaacagcatctatggttgcgaagttagcaaagaaccggtgtttaaattctatgccgatctgctgtatatccgcaaaaatctggcagttctggaacacaaaaataacctgccgagcaatcaagaagagttcatctgcaaaatcaacaacacctttgaaaacattgtgctgccgtataaaatcagccagttcgaaacctacaaaaaagatattctggcctggattaacgatggccatgatcataaaaagtataccgatgcaaaacagcagctgggttttattcgtggtggtctgaaaggtcgtattaaagcagaagaagttagccagaaagacaagtacggtaaaatcaaaagctattatgagaacccgtacaccaaactgaccaacgaatttaagcagattagcagcacatatggcaaaacctttgcagaactgcgcgacaaattcaaagaaaaaaacgagatcaccaaaatcacccactttggcattatcatcgaagataaaaaccgtgatcgttatctgctggcaagtgagctgaaacatgagcagattaatcatgttagcaccatcctgaacaaactggataaaagctcagaattcattacctatcaggtgaaaagcctgaccagtaaaaccctgattaaactgatcaaaaaccataccaccaaaaagggtgcgattagcccgtatgcagattttcataccagcaaaaccggcttcaacaaaaatgagatcgagaaaaactgggacaactataaacgtgaacaggtcctggttgagtatgttaaagattgtctgaccgatagcaccatggccaaaaatcagaattgggcagaatttggctggaactttgaaaagtgtaacagctatgaagatatcgagcacgagattgatcagaaaagctatctgctgcagagcgataccattagcaaacagagcattgcaagcctggttgaaggtggttgtctgctgctgccgattattaaccaggatattaccagtaaagagcgcaaagacaaaaaccagttcagcaaagattggaaccatatctttgaaggcagcaaagaatttcgtctgcatccggaatttgcagttagctatcgtaccccgattgaaggttatccggttcagaaacgttatggtcgtctgcagtttgtttgtgcatttaatgcccatattgttccgcagaatggcgaatttatcaacctgaaaaagcagattgagaacttcaacgatgaggatgtgcagaaacgtaatgtgaccgaatttaacaaaaaagtgaatcatgccctgagcgacaaagaatatgttgtgattggtattgatcgcggtctgaaacaactggcgaccctgtgtgttctggataaacgtggtaaaattctgggcgatttcgagatctacaagaaagaatttgttcgtgccgaaaaacgtagcgaaagccattgggaacacacccaggcagaaacccgtcatattctggatctgagcaatctgcgtgttgaaaccacaattgaaggtaaaaaagtgctggttgatcagagtctgaccctggttaaaaagaatcgtgatacaccggatgaagaagccaccgaagaaaataaacagaagatcaaactgaagcagctgagctatattcgtaaactgcagcataaaatgcagaccaatgaacaggatgttctggacctgattaataacgaaccgagtgatgaggaattcaaaaaacgtattgaaggcctgatttccagctttggtgaaggtcagaaatatgcggatctgcctattaataccatgcgcgaaatgattagcgatctgcagggtgttattgcacgtggtaataatcagaccgagaagaacaaaatcattgaactggatgcagccgataatctgaaacagggtattgttgcaaacatgattggcatcgtgaactacatctttgccaaatacagctacaaagcctatatcagcctggaagatctgagccgtgcatatggtggtgcaaaaagcggttatgatggtcgctatctgccgagtaccagccaggacgaagatgtggattttaaagaacagcagaatcagatgctggcaggtctgggcacctatcagtttttcgaaatgcaactgctgaagaagctgcagaaaattcagagtgataataccgttctgcgctttgttccggcatttcgtagcgcagataactatcgtaatattctgcgtctggaagaaaccaagtataaaagcaaaccgtttggcgtggtgcactttattgatccgaaatttacgagcaaaaaatgtccggtttgtagcaaaaccaatgtgtaccgcgataaagatgacattctggtttgtaaagaatgcggttttcgtagtgatagccaactgaaagaacgcgaaaacaacatccattatattcacaatggtgatgacaacggtgcctatcatattgcactgaaaagcgtggaaaatctgatccagatgaaataatggtctagaggtcgaaattcaaattgtgagcggataacaatttgaattttctgtatgaggttttgctaaacaactttcaacagtttcagtggagtgagaatagaaaggaacaactaaaggaattgcgaataataattttttcacgttgaaaatctccaaaaaaaaaggctccaaaaggagcctttaattgtatcggtttatcagcttgctttcgaggtgaattttgaccctctagcgaaaatgcaagagcaaagacgaaaacatgccacacatgaggaataccgattctctcattaacatattcaggccagttatctgggcttaaaagcagaagtccaacccagataacgatcatatacatggttctctccagaggttcattactgaacactcgtccgagaataacgagtggatcccctccaattcgccctatagtgagtcgtattacgcgcgctcactggccgtcgttttacaacgtcgtgactgggaaaaccctggcgttacccaacttaatcgccttgcagcacatccccctttcgccagctggcgtaatagcgaagaggcccgcaccgatcgcccttcccaacagttgcgcagcctgaatggcgaatggaaattgtaagcgttaatattttgttaaaattcgcgttaaatttttgttaaatcagctcattttttaaccaataggccgactgcgatgagtggcagggcggggcgtaatttttttaaggcagttattggtgcccttaaacgcctggtgctacgcctgaataagtgataataagcggatgaatggcagaaattcgaaagcaaattcgacccggtcgtcggttcagggcagggtcgttaaatagccgcttatgtctattgctggtttaccggtttattgactaccggaagcagtgtgaccgtgtgcttctcaaatgcctgaggccagtttgctcaggctctccccgtggaggtaataattgacgatatgatcatttattctgcctcccagagcctgataaaaacggtgaatccgttagcgaggtgccgccggcttccattcaggtcgaggtggcccggctccatgcaccgcgacgcaacgcggggaggcagacaaggtatagggcggcgaggcggctacagccgatagtctggaacagcgcacttacgggttgctgcgcaacccaagtgctaccggcgcggcagcgtgacccgtgtcggcggctccaacggctcgccatcgtccagaaaacacggctcatcgggcatcggcaggcgctgctgcccgcgccgttcccattcctccgtttcggtcaaggctggcaggtctggttccatgcccggaatgccgggctggctgggcggctcctcgccggggccggtcggtagttgctgctcgcccggatacagggtcgggatgcggcgcaggtcgccatgccccaacagcgattcgtcctggtcgtcgtgatcaaccaccacggcggcactgaacaccgacaggcgcaactggtcgcggggctggccccacgccacgcggtcattgaccacgtaggccgacacggtgccggggccgttgagcttcacgacggagatccagcgctcggccaccaagtccttgactgcgtattggaccgtccgcaaagaacgtccgatgagcttggaaagtgtcttttggctgaccaccacggcgttctggtggcccatctgcgccacgaggtgatgcagcagcattgccgccgtgggtttcctcgcaataagcccggcccacgcctcatgcgctttgcgttccgtttgcacccagtgaccgggcttgttcttggcttgaatgccgatttctctggactgcgtgg

SEQ ID NO: 36 - DNA, 10542 bp, synthetic construct
  misc_feature 1..10542: note = CRISPR/SeqID63_Coli vector system
  source 1..10542: mol_type = other DNA
ccatgcttatctccatgcggtagggtgccgcacggttgcggcaccatgcgcaatcagctgcaacttttcggcagcgcgacaacaattatgcgttgcgtaaaagtggcagtcaattacagattttctttaacctacgcaatgagctattgcggggggtgccgcaatgagctgttgcgtaccccccttttttaagttgttgatttttaagtctttcgcatttcgccctatatctagttctttggtgcccaaagaagggcacccctgcggggttcccccacgccttcggcgcggctccccctccggcaaaaagtggcccctccggggcttgttgatcgactgcgcggccttcggccttgcccaaggtggcgctgcccccttggaacccccgcactcgccgccgtgaggctcggggggcaggcgggcgggcttcgccttcgactgcccccactcgcataggcttgggtcgttccaggcgcgtcaaggccaagccgctgcgcggtcgctgcgcgagccttgacccgccttccacttggtgtccaaccggcaagcgaagcgcgcaggccgcaggccggaggcttttccccagagaaaattaaaaaaattgatggggcaaggccgcaggccgcgcagttggagccggtgggtatgtggtcgaaggctgggtagccggtgggcaatccctgtggtcaagctcgtgggcaggcgcagcctgtccatcagcttgtccagcagggttgtccacgggccgagcgaagcgagccagccggtggccgctcgcggccatcgtccacatatccacgggctggcaagggagcgcagcgaccgcgcagggcgaagcccggagagcaagcccgtagggcgccgcagccgccgtaggcggtcacgactttgcgaagcaaagtctagtgagtatactcaagcattgagtggcccgccggaggcaccgccttgcgctgcccccgtcgagccggttggacaccaaaagggaggggcaggcatggcggcatacgcgatcatgcgatgcaagaagctggcgaaaatgggcaacgtggcggccagtctcaagcacgcctaccgcgagcgcgagacgcccaacgctgacgccagcaggacgccagagaacgagcactgggcggccagcagcaccgatgaagcgatgggccgactgcgcgagttgctgccagagaagcggcgcaaggacgctgtgttggcggtcgagtacgtcatgacggccagcccggaatggtggaagtcggccagccaagaacagcaggcggcgttcttcgagaaggcgcacaagtggctggcggacaagtacggggcggatcgcatcgtgacggccagcatccaccgtgacgaaaccagcccgcacatgaccgcgttcgtggtgccgctgacgcaggacggcaggctgtcggccaaggagttcatcggcaacaaagcgcagatgacccgcgaccagaccacgtttgcggccgctgtggccgatctagggctgcaacggggcatcgagggcagcaaggcacgtcacacgcgcattcaggcgttctacgaggccctggagcggccaccagtgggccacgtcaccatcagcccgcaagcggtcgagccacgcgcctatgcaccgcagggattggccgaaaagctgggaatctcaaagcgcgttgagacgccggaagccgtggccgaccggctgacaaaagcggttcggcaggggtatgagcctgccctacaggccgccgcaggagcgcgtgagatgcgcaagaaggccgatcaagcccaagagacggcccgagaccttcgggagcgcctgaagcccgttctggacgccctggggccgttgaatcgggatatgcaggccaaggccgccgcgatcatcaaggccgtgggcgaaaagctgctgacggaacagcgggaagtccagcgccagaaacaggcccagcgccagcaggaacgcgggcgcgcacatttccccgaaaagtgccacctgaaccccagagtcccgctcagaagaactcgtcaagaaggcgatagaaggcgatgcgctgcgaatcgggagcggcgataccgtaaagcacgaggaagcggtcagcccattcgccgccaagctcttcagcaatatcacgggtagccaacgctatgtcctgatagcggtccgccacacccagccggccacagtcgatgaatccagaaaagcggccattttccaccatgatattcggcaagcaggcatcgccatgggtcacgacgagatcctcgccgtcgggcatccgcgccttgagcctggcgaacagttcggctggcgcgagcccctgatgctcttcgtccagatcatcctgatcgacaagaccggcttccatccgagtacgtgctcgctcgatgcgatgtttcgcttggtggtcgaatgggcaggtagccggatcaagcgtatgcagccgccgcattgcatcagccatgatggatactttctcggcaggagcaaggtgagatgacaggagatcctgccccggcacttcgcccaatagcagccagtcccttcccgcttcagtgacaacgtcgagcacagctgcgcaaggaacgcccgtcgtggccagccacgatagccgcgctgcctcgtcttggagttcattcagggcaccggacaggtcggtcttgacaaaaagaaccgggcgcccctgcgctgacagccggaacacggcggcatcagagcagccgattgtctgttgtgcccagtcatagccgaatagcctctccacccaagcggccggagaacctgcgtgcaatccatcttgttcaatcatgcgaaacgatcctcatcctgtctcttgatcagatcttgatcccctgcgccatcagatccttggcggcaagaaagccatccagtttactttgcagggcttcccaaccttaccagagggcgccccagctggcaattccggttcgcttgctgtccataaaaccgcccagtctagctatcgccatgtaagcccactgcaagctacctgctttctctttgcgcttgcgttttcccttgtccagatagcccagtagctgacattcatccggggtcagcaccgtttctgcggactggctttctacgtgttccgcttcctttagcagcccttgcgccctgagtgcttgcggcagcgtgaagctagcataaaacgaaaggcccagtctttcgactgagcctttcgttttatttgatgcctggcagttccctactctcgcatggggagaccccacactaccatcggcgctacggcgtttcacttctgagttcggcatggggtcaggtgggaccaccgcgctactgccgccaggcaaaaaaaaaagtcccggttgagtacatcgcaggatctacaacagtagaaattcgacctcattctattagactctcgtttggattgcaactggtctattttcctcttttgtttgatagaaaatcataaaaggatttgcagactacgggcctaaagaactaaaaaatctatctgtttcttttcattctctgtattttttatagtttctgttgcatgggctgcataatgtgcctgtcaaatggacgaagcagggattctgcaaaccctatgctactccgtcaagccgtcaattgtctgattcgttaccaattatgacaacttgacggctacatcattcactttttcttcacaaccggcacggaactcgctcgggctggccccggtgcattttttaaatacccgcgagaaatagagttgatcgtcaaaaccaacattgcgaccgacggtggcgataggcatccgggtggtgctcaaaagcagcttcgcctggctgatacgttggtcctcgcgccagcttaagacgctaatccctaactgctggcggaaaagatgtgacagacgcgacggcgacaagcaaacatgctgtgcgacgctggcgatatcaaaattgctgtctgccaggtgatcgctgatgtactgacaagcctcgcgtacccgattatccatcggtggatggagcgactcgttaatcgcttccatgcgccgcagtaacaattgctcaagcagatttatcgccagcagctccgaatagcgcccttccccttgcccggcgttaatgatttgcccaaacaggtcgctgaaatgcggctggtgcgcttcatccgggcgaaagaaccccgtattggcaaatattgacggccagttaagccattcatgccagtaggcgcgcggacgaaagtaaacccactggtgataccattcgcgagcctccggatgacgaccgtagtgatgaatctctcctggcgggaacagcaaaatatcacccggtcggcaaacaaattctcgtccctgatttttcaccaccccctgaccgcgaatggtgagattgagaatataacctttcattcccagcggtcggtcgataaaaaaatcgagataaccgttggcctcaatcggcgttaaacccgccaccagatgggcattaaacgagtatcccggcagcaggggatcattttgcgcttcagccatacttttcatactcccgccattcagagaagaaaccaattgtccatattgcatcagacattgccgtcactgcgtcttttactggctcttctcgctaaccaaaccggtaaccccgcttattaaaagcattctgtaacaaagcgggaccaaagccatgacaaaaacgcgtaacaaaagtgtctataatcacggcagaaaagtccacattgattatttgcacggcgtcacactttgctatgccatagcatttttatccataagattagcggatcctacctgacgctttttatcgcaactctctactgtttctccatacccgttttttggtaccgggccccccctcgagtttattttaggaggcaaaaatgaaaagctttgaaaacagctgccagattagcaaaaccctgcgttttggtgcaaccctgaaagaggataaaaagaaatgcaaaagccacgaggaactgcaagaatttgtggatattagctataaaaccatgaaaagcagcgcaaccattgcagaaagcctgaatgaaattgaactggtgaaaaagtgcgaacgctgctatagcgaaatcatcaaatttcatgaagcctggggtcagatttattgtcgtaccgatcagattgccgtgtacaaagatttttatcgtcagctggcacgtaaagcccgttttgatgttggtgatcagaatagccagctgattaccctgagcagcctgagtagcaaacataatgtttatcagggtctgaaacgcagccagcatattaccaattattggaaagataacattgcccgtcagaaaagcttcctgaaagattttagccagcagctgcatcagtataaacgtgcactggaaaatagcgataaagcacataccaaaccgaacctgatcaacttcaataaaacctttagcattctggccaacctggtgaacgaaattgttattccgctgagcaatggtgcaattagctttccgaatatcagcaaactggaagatggtgaagaaagccgtcatctgattgaatttgccctgaatgattatagcgatctggttggtagcattggcgaactgaaagatgcaattgccaccaatggtggttataccccgtttgcaaaagttaccctgaaccattataccgcagaacagaaaccgcatgtgttcaaaaatgatatcgatgccaaaatccgtgagctgaaactgatcgaactggttgagaaactgaaaaacaaaaccagcaagcagatcgaagagtacttcagcaaattcgacaagttcaaaatctatgatgatcgcaaccagagcgtgattattcgtacccagtgctttaaatacaaaccgattccgtttctggtgaaacatgaactggccaaatatatcgccgaagatgaagatgcagttctgaaagttctggatgccattggtgcgacccgtagtccggcacatgattatgcacataatgaagatgtgttcgacctgaaacactatccgattaaagtggcatttgattatgcctgggaacagctggcaaatggtgtgtataccaccgtgagctttccggaagaaaaatgtcgtgaatatctgaacgccatttatggttgcgaagttaccaaagaaccggtgttcaaattttacgccgatctgctgtatattcgcaaaaatctggccgttctggaacacaaaaataacctgccgagcaatccggaagagtttatttgcaaaatcgaaaacaccttcgagaaaatcgtgctgccgtataaaatcaaagagttcgaaacctacaaaaaggccattctgacctggattaatgatggtcgtggtcatgagaaatataccgatagcaaacgtgaactgggtctgattcgtggtggtctgaaaggtcgtattggtgcacagaaaatgttccgcaaaaataagaaaggtgagctgatcccgtattatgaaaacccgtataccaaactgaccaacgagtttaaaaacatcagcagcagctatggcaaaacctttgccgaactgcgtgataagtttaaagagaaaagcgagatcacgaagatcacccattttggtatcatcatcgaggacaataacaaagatcgttatctgctggccaatggtctgcagcatgataatacagatcagagcaatacccaggttgaagcaattctgggtaaactgaataccagcctggaatttaccacctatcaggttaaaagcctgaccagcaaaatcctgattaagctgattaaaaaccatacgaccagtccgaatgcaaaaagcccgtatgcagattttcatacctccaaaattcatgtggactggaccaaaatcaagaaagagtgggatacctataaaagcaaccattcactgctgcagtatgtgaaagattgtctgaccaatagcaccatggccaaaaatcagaattgggcagaatttggctgggatttagaaagctgtaatagctatgaagccatcgaacatgagattgaccagaaaagttatatcctgcagaaacacacaattagcaaagccagcattaaatccctggttgaaaatggttgtctgctgctgccgattgtgaatcaggatattaccagccagggtcgcaaagataaaaaccagtttagcaaagattggaagcagatcttcgaggatagcaaagaatatcgtctgcatccggaatttgcagttagctatcgtaccccgatcaaagattatccgaaagataaacgttatggtcgcctgcagtttatctgtgcctttaactgtgaaatcattccgcagaatggcgaatttatcaacctgaaaaagcagattgagaacttcaacgatgaggatatccagaaaaataacgtggccgaattcaacaacaaagtgaatgaagccctgctgggtaaagaatatgttgtgattggtattgatcgtggcctgaaacaactggcaaccctgtgtgttctgaataaacgtggtaaaattctgggcgatttcgagatctacaagaaagaattcgttcgtaccgaaaaccgcagcaaaaactattggaaacacaccctggcagaaacccgtcatattctggatctgagcaatctgcgtgttgaaaccaccgttgaagataataaagtgctggttgatcagagtctgaccctggttaaaaagaatcgtgatacaccggatgaaaaagccaccgaagaaaatcgccagaaaatcaaactgaaacagctgagctatattcgtaagctgcagtacgcaatgcagaccaatgaacaggcagtgctggatctgctgaaagataatagtgatgatgaagagttcaaaaagcgtgtggaaggtgttattagcccgtttggtgaaggtcaagaatatgcggatctgccgatcgataccatgcgtgcaatgattcaggatctgcagggtgttattgccaaaggtaataaacagaccgagaaaaacaagatcattgagctggatgcagcggatagtctgaaacagggtgttgtggcaaatatgattggtgtggttaactttatcctggcgaaattcaactatgaagcgtatgttagcctggaagatctgagccgtgcatataatgttgccaaaagcggttatgatggacgctatctgccgagtaccagtcaggatccggatatggattttaaagaacagcagaatcagatgctggcaggtctgggtacatatcagtttttcgaaattcagctgctgaagaagctgcagaaaattcagagtaataataccgtgctgcgctttgttccggcatttcgtagcgcagataactatcgcaatattatcaagctgaacccgaaatatgataacaccgagtatgttcataaaccgtttggcattgtgcatttcattgatcctaaagacaccagcagcaaatgtccggtttgtggtaaaaccggcaaaaagaatgttgatcgcaatgagaagaagaacaatatcctgctgtgcaaagcatgtggttttcgtaccgtgtgggaattaaaacagccggaaaacattaaaagcgagggctattgttttagcgaagatgagattcagaaaaccatcaaaaacaaccagaaacaaatggaaatcaaaaagctgagcgacaaaaacatccactacattcataacggtgatgataacggtgcatatcatattgcactgaaaagcgtggaaaacctgaagcacaaagaataatggtctagaggtcgaaattcaaattgtgagcggataacaatttgaattttctgtatgaggttttgctaaacaactttcaacagtttcagtggagtgagaatagaaaggaacaactaaaggaattgcgaataataattttttcacgttgaaaatctccaaaaaaaaaggctccaaaaggagcctttaattgtatcggtttatcagcttgctttcgaggtgaattttgaccctctagcgaaaatgcaagagcaaagacgaaaacatgccacacatgaggaataccgattctctcattaacatattcaggccagttatctgggcttaaaagcagaagtccaacccagataacgatcatatacatggttctctccagaggttcattactgaacactcgtccgagaataacgagtggatcccctccaattcgccctatagtgagtcgtattacgcgcgctcactggccgtcgttttacaacgtcgtgactgggaaaaccctggcgttacccaacttaatcgccttgcagcacatccccctttcgccagctggcgtaatagcgaagaggcccgcaccgatcgcccttcccaacagttgcgcagcctgaatggcgaatggaaattgtaagcgttaatattttgttaaaattcgcgttaaatttttgttaaatcagctcattttttaaccaataggccgactgcgatgagtggcagggcggggcgtaatttttttaaggcagttattggtgcccttaaacgcctggtgctacgcctgaataagtgataataagcggatgaatggcagaaattcgaaagcaaattcgacccggtcgtcggttcagggcagggtcgttaaatagccgcttatgtctattgctggtttaccggtttattgactaccggaagcagtgtgaccgtgtgcttctcaaatgcctgaggccagtttgctcaggctctccccgtggaggtaataattgacgatatgatcatttattctgcctcccagagcctgataaaaacggtgaatccgttagcgaggtgccgccggcttccattcaggtcgaggtggcccggctccatgcaccgcgacgcaacgcggggaggcagacaaggtatagggcggcgaggcggctacagccgatagtctggaacagcgcacttacgggttgctgcgcaacccaagtgctaccggcgcggcagcgtgacccgtgtcggcggctccaacggctcgccatcgtccagaaaacacggctcatcgggcatcggcaggcgctgctgcccgcgccgttcccattcctccgtttcggtcaaggctggcaggtctggttccatgcccggaatgccgggctggctgggcggctcctcgccggggccggtcggtagttgctgctcgcccggatacagggtcgggatgcggcgcaggtcgccatgccccaacagcgattcgtcctggtcgtcgtgatcaaccaccacggcggcactgaacaccgacaggcgcaactggtcgcggggctggccccacgccacgcggtcattgaccacgtaggccgacacggtgccggggccgttgagcttcacgacggagatccagcgctcggccaccaagtccttgactgcgtattggaccgtccgcaaagaacgtccgatgagcttggaaagtgtcttttggctgaccaccacggcgttctggtggcccatctgcgccacgaggtgatgcagcagcattgccgccgtgggtttcctcgcaataagcccggcccacgcctcatgcgctttgcgttccgtttgcacccagtgaccgggcttgttcttggcttgaatgccgatttctctggactgcgtgg

SEQ ID NO: 37 - DNA, 3696 bp, synthetic construct
  misc_feature 1..3696: note = E. Coli codonoptimized NT sequences of BEC10
  source 1..3696: mol_type = other DNA
atgaaaagctttgaaaacagctgccagattagcaaaaccctgcgttttggtgcaaccctgaaagaggataaaaagaaatgtaaaagccacctggaactgcaagaatttgtggatattagctacaagaccctgaaaagcagcgcaaccattgcagaaagcctgaatgaaattgagctggtgaaaaaatgcgaacgctgctatagcgaaatcatcaaatttcatgaagcctggggtcagatttattgtcgtaccaatcagattgccgtgtacaaagattggtatcgtcagctggcacgtaaagcacgttttgatgttggtgatcagaatagccagctgattaccctgagcagcctgagtagcaaacataatgtttatcagggtctgaaacgcagccagcatattaccaattattggaaagataacattgcccgtcagaaaagcttcctgaaagattttagccagcagctgaaacagtataaacgtgcactggaaaatagcgataaagcacataccaaaccgaacctgatcaacttcaataaaacctttagcattctggccaacctggtgaacgaaattgttattccgctgagcaatggtgcaattagctttccgaatatcagcaaactggaagatggtgaagaaagccgtcatctgattgaatttgccctgaatgattatagcgatctggttggtagcattggcgaactgaaagatgcaattgccaccaatggtggttataccccgtttgcaaaagttaccctgaaccattataccgcagaacagaaaccgcatgtgttcaaaaatgatatcgatgccaaaatccgtgagctgaaactgattgaactggttgagaaactgaaaaacaaaaccagcaagcagatcgaagagtacttcagcaaattcgacaagttcaaaatctatgatgatcgcaacatcagcgtgattattcgtacccagtgctttaaatacaaaccgattccgtttctggtgaaacatgaactggccaaatatatcgccgaagatgaagatgcagttctgaaagttctggatgccattggtgcgacccgtagtccggcacatgattatgcacataatgaagatgtgttcgatctgaaccactatccgattaaagtggcatttgattatgcctgggaacagctggcaaatggtgtgtataccaccgtgacctttccgaaagaacagtgtgaaaaatatctgaaggatgtgtttgattgcgaggttagcaaagaaccggtgtttaaattctatgccgatctgctgtatatccgcaaaaatctggccgttctggaacataaaaacaatctgccgagcaaccaagaagagttcatttgcaaaatcaacaacaccttcgaaaacatcgtgctgccgtataaaatcaaagagttcgaaacctacaaaaaagacatcctggcctggattaatgatggtcgtggtcatgagaaatataccgatgcaaaacagcagctgggttttattcgtggtggtctgaaaggtcgtattaaagcccagaaaatgttccgcaaagataagtacggtaagatcaaaagctattatgagaacccgtataccaaactgaccaacgaatttaagcagatcagcagcacctatggcaaaacctttgccgaactgcgtgataagtttaaagagaagaacaacatcaccaaaatcacccactttggcatcatcatcgaggataataacaaagatcgttatctgctggccaatggtctgcagcatgagcagattaatcatgttgaagcaattctgggcaaactgaataccagcagcgaatttatcacctatcaggttaaaagcctgaccagtaaaaccctgattaagctgattaaaaaccataccaccaaaaagggtgcgattagcccgtatgcagattttcataccagcaaaattcatgtggactggacgaaaatcaaaaaagagtgggataactataagcgcgaacaggttctgctgcagtatgttaaagattgtctgaccgatagcaccatggccaaaaatcagaattgggcagaatttggctggaactttgaaaaatgcaacagctatgaagatatcgagcacgagattgaccagaaaagttatatcctgcagaaacacaccatctccaaacagagcattgcaagcctggttgaaggtggttgtctgctgctgccgattattaaccaggatattacctcacagggtcgcaaagacaaaaaccagtttagtaaagattggaagcagatctttgaaggcagcaaagaatttcgtctgcatccggaatttgcagttagctatcgtaccccgatcaaagattatccgaaagataaacgttatggtcgcctgcagtttgtttgtgcctttaactgtgaaatcattccgcagaatggcgaattcatcaatctgaaaaagcagattgagaacttcaacgatgaggatgcacagaaagaagccgttgaagaattcaacaaaaaagtgaatcatgccctgctgggcaaagaatatgttgtgattggtattgatcgtggcctgaaacaactggcaaccctgtgtgttctggataaacgtggtaaaatcctgggcgattttgagatctacaagaaagaattcgttcgtgccgaaaaacgcagcaaaaactattggaaacacacactggcagaaacccgtcatattctggatctgagcaatctgcgtgttgaaaccacaatcgaagataacaaagtgctggttgatcagagtctgaccctggttaaaaagaatcgtgatacaccggatgaagaagccaccgaagaaaataaacagaagatcaaactgaagcagctgagctatattcgtaaactgcagcataaaatgcagaccaatgaacaggatgttctggacctgattaataacgaaccgagcgacgaagaatttaagaaacgtattgaaggtctgattagcagctttggtgaaggtcagaaatatgcggatctgcctattaataccatgcgcgaaatgattagtgatctgcagggtgttattgcccgtggtaataatcagacagagaaaaacaagatcatcgaactggatgcagccgataatctgaaacagggtattgttgcaaacatgattggcatcgtgaactacatctttgccaaatacagctacaaagcctatatcagcctggaagatctgagccgtgcatatggtggtgcaaaaagcggttatgatggacgctatctgccgtcaaccagccaggacgaagatgtggattttaaagaacagcagaatcagatgctggcaggtctgggtacatatcagttttttgaaatgcagctgctgaagaagctgcagaaaattcagagcgataataccgttctgcgctttgttccggcatttcgtagcgcagataactatcgcaatattatcaagctggaagaaaccaaatacaaaagcaaaccgtttggcgtggtgcactttattgatccgaaatttacgagcaaaaaatgtccggtttgcagcaaaaccaatgtgtatcgtgataaagatgacattctggtgtgtaaagaatgcggttttcgtagtgatagtcagctgaaagaacgcgaaaacaacatccactatattcataatggtgatgacaacggtgcctatcatattgcactgaaaagcgtggaaaatctgatccagatgaaataa

SEQ ID NO: 38 - DNA, 85 bp, synthetic construct
  misc_feature 1..85: note = AraBAD promotor sequences
  source 1..85: mol_type = other DNA
ggcgtcacactttgctatgccatagcatttttatccataagattagcggatcctacctgacgctttttatcgcaactctctactg

SEQ ID NO: 39 - DNA, 177 bp, synthetic construct
  misc_feature 1..177: note = Fdt terminator sequence
  source 1..177: mol_type = other DNA
aattttctgtatgaggttttgctaaacaactttcaacagtttcagtggagtgagaatagaaaggaacaactaaaggaattgcgaataataattttttcacgttgaaaatctccaaaaaaaaaggctccaaaaggagcctttaattgtatcggtttatcagcttgctttcgaggtgaa

SEQ ID NO: 40 - DNA, 164 bp, synthetic construct
  misc_feature 1..164: note = SacB RNA polymerase III promotor sequence
  source 1..164: mol_type = other DNA
gcccatgcaacagaaactataaaaaatacagagaatgaaaagaaacagatagattttttagttctttaggcccgtagtctgcaaatccttttatgattttctatcaaacaaaagaggaaaatagaccagttgcaatccaaacgagagtctaatagaatgaggtc

SEQ ID NO: 41 - DNA, 169 bp, synthetic construct
  misc_feature 1..169: note = RrnB terminator sequence
  source 1..169: mol_type = other DNA
tttgcctggcggcagtagcgcggtggtcccacctgaccccatgccgaactcagaagtgaaacgccgtagcgccgatggtagtgtggggtctccccatgcgagagtagggaactgccaggcatcaaataaaacgaaaggctcagtcgaaagactgggcctttcgttttat

SEQ ID NO: 42 - DNA, 24 bp, synthetic construct
  misc_feature 1..24: note = RpoB target-specific spacer sequences
  source 1..24: mol_type = other DNA
cctgcgatgtactcaaccgggact